European Patent Specification EP 3 505 179 B1, published April 8, 2026. Title: CHIMERIC FACTOR VIII POLYPEPTIDES AND USES THEREOF. Applicant: Biogen Idec MA Inc. Application To be assigned. The sequence listing filed with the application follows.

SEQUENCE LISTING (114 sequences)

SEQ ID NO: 1 - DNA, 16842 bp, Homo sapiens
atgattcctgccagatttgccggggtgctgcttgctctggccctcattttgccagggaccctttgtgcagaaggaactcgcggcaggtcatccacggccctactaaggacggtctaaacggccccacgacgaacgagaccgggagtaaaacggtccctgggaaacacgtcttccttgagcgccgtccagtaggtgccggggatgcagccttttcggaagtgacttcgtcaacacctttgatgggagcatgtacagctttgcgggatactgcagttacctcctggcagggggctgccagaactacgtcggaaaagccttcactgaagcagttgtggaaactaccctcgtacatgtcgaaacgccctatgacgtcaatggaggaccgtcccccgacggtcttacgctccttctcgattattggggacttccagaatggcaagagagtgagcctctccgtgtatcttggggaattttttgacatccatttgtttgtcaatggttgcgaggaagagctaataacccctgaaggtcttaccgttctctcactcggagaggcacatagaaccccttaaaaaactgtaggtaaacaaacagttaccaaccgtgacacagggggaccaaagagtctccatgccctatgcctccaaagggctgtatctagaaactgaggctgggtactacaagctgtccggtgaggccttggcactgtgtccccctggtttctcagaggtacgggatacggaggtttcccgacatagatctttgactccgacccatgatgttcgacaggccactccggaatggctttgtggccaggatcgatggcagcggcaactttcaagtcctgctgtcagacagatacttcaacaagacctgcgggctgtgtggcaactttaacattaccgaaacaccggtcctagctaccgtcgccgttgaaagttcaggacgacagtctgtctatgaagttgttctggacgcccgacacaccgttgaaattgtactttgctgaagatgactttatgacccaagaagggaccttgacctcggacccttatgactttgccaactcatgggctctgagcagtggagaacagtggtgtgaaacgacttctactgaaatactgggttcttccctggaactggagcctgggaatactgaaacggttgagtacccgagactcgtcacctcttgtcaccacagaacgggcatctcctcccagcagctcatgcaacatctcctctggggaaatgcagaagggcctgtgggagcagtgccagcttctgaagagcacctcggtgtcttgcccgtagaggagggtcgtcgagtacgttgtagaggagacccctttacgtcttcccggacaccctcgtcacggtcgaagacttctcgtggagccacattgcccgctgccaccctctggtggaccccgagccttttgtggccctgtgtgagaagactttgtgtgagtgtgctggggggctggagtgcgcctgccctgcaacgggcgacggtgggagaccacctggggctcggaaaacaccgggacacactcttctgaaacacactcacacgaccccccgacctcacgcggacgggacgcctcctggagtacgcccggacctgtgcccaggagggaatggtgctgtacggctggaccgaccacagcgcgtgcagcccagtgtgccctgctggtatggagggaggacctcatgcgggcctggacacgggtcctcccttaccacgacatgccgacctggctggtgtcgcgcacgtcgggtcacacgggacgaccatacctctataggcagtgtgtgtccccttgcgccaggacctgccagagcctgcacatcaatgaaatgtgtcaggagcgatgcgtggatggctgcagctgccctgaggatatccgtcacacacaggggaacgcggtcctggacggtctcggacgtgtagttactttacacagtcctcgctacgcacctaccgacgtcgacgggactccgacagctcctggatgaaggcctctgcgtggagagcaccgagtgtccctgcgtgcattccggaaagcgctaccctcccggcacctccctctctcgagactgctgtcgaggacctacttccggagacgcacctctcgtggctcacagggacgcacgtaaggcctttcgcgatgggagggccgtggagggagagagctctgaccaacacctgcatttgccgaaacagccagtggatctgcagcaatgaagaatgtccaggggagtgccttgtcactggtcaatcccacttcaagagctttgacgttgtggacgtaaacggctttgtcggtcacctagacgtcgttacttcttacaggtcccctcacggaacagtgaccagttagggtgaagttctcgaaactgaacagatacttcaccttcagtgggatctgccagtacctgctggcccgggattgccaggaccactccttctccattgtcattgagactgtccagtgtgctgttgtctatgaagtggaagtcaccctagacggtcatggacgaccgggccctaacggtcctggtgaggaagaggtaacagtaactctgacaggtcacacgacatgaccgcgacgctgtgtgcacccgctccgtcaccgtccggctgcctggcctgcacaacagccttgtgaaactgaagcatggggcaggagttgccatggatactggcgctgcgacacacgtgggcgaggcagtggcaggccgacggaccggacgtgttgtcggaacactttgacttcgtaccccgtcctcaacggtaccttggccaggacatccagctccccctcctgaaaggtgacctccgcatccagcatacagtgacggcctccgtgcgcctcagctacggggaggacctgcagatgaccggtcctgtaggtcgagggggaggactttccactggaggcgtaggtcgtatgtcactgccggaggcacgcggagtcgatgcccctcctggacgtctacgactgggatggccgcgggaggctgctggtgaagctgtcccccgtctatgccgggaagacctgcggcctgtgtgggaattacaatggcaaccagggcgacgctgaccctaccggcgccctccgacgaccacttcgacagggggcagatacggcccttctggacgccggacacacccttaatgttaccgttggtcccgctgcacttccttaccccctctgggctggcrgagccccgggtggaggacttcgggaacgcctggaagctgcacggggactgccaggacctgcagaagcagcacagtgaaggaatgggggagacccgaccgyctcggggcccacctcctgaagcccttgcggaccttcgacgtgcccctgacggtcctggacgtcttcgtcgtgtccgatccctgcgccctcaacccgcgcatgaccaggttctccgaggaggcgtgcgcggtcctgacgtcccccacattcgaggcctgccatcgtgccgtcagcgctagggacgcgggagttgggcgcgtactggtccaagaggctcctccgcacgcgccaggactgcagggggtgtaagctccggacggtagcacggcagtcgccgctgccctacctgcggaactgccgctacgacgtgtgctcctgctcggacggccgcgagtgcctgtgcggcgccctggccagctatgccgcggcctgcgggcgacgggatggacgccttgacggcgatgctgcacacgaggacgagcctgccggcgctcacggacacgccgcgggaccggtcgatacggcgccggacgccggggagaggcgtgcgcgtcgcgtggcgcgagccaggccgctgtgagctgaactgcccgaaaggccaggtgtacctgcagtgcgggaccccctgcaacctgcccctctccgcacgcgcagcgcaccgcgctcggtccggcgacactcgacttgacgggctttccggtccacatggacgtcacgccctgggggacgttggagacctgccgctctctctcttacccggatgaggaatgcaatgaggcctgcctggagggctgcttctgccccccagggctctacatggatgagaggggggacctggacggcgagagagagaatgggcctactccttacgttactccggacggacctcccgacgaagacggggggtcccgagatgtacctactctcccccctgtgcgtgcccaaggcccagtgcccctgttactatgacggtgagatcttccagccagaagacatcttctcagaccatcacaccatgtgctactgtgaggatgacgcacgggttccgggtcacggggacaatgatactgccactctagaaggtcggtcttctgtagaagagtctggtagtgtggtacacgatgacactcctacgcttcatgcactgtaccatgagtggagtccccggaagcttgctgcctgacgctgtcctcagcagtcccctgtctcatcgcagcaaaaggagcctatcctgcgaagtacgtgacatggtactcacctcaggggccttcgaacgacggactgcgacaggagtcgtcaggggacagagtagcgtcgttttcctcggataggactcggccccccatggtcaagctggtgtgtcccgctgacaacctgcgggctgaagggctcgagtgtaccaaaacgtgccagaactatgacctggagtgcatgagccggggggtaccagttcgaccacacagggcgactgttggacgcccgacttcccgagctcacatggttttgcacggtcttgatactggacctcacgtacagcatgggctgtgtctctggctgcctctgccccccgggcatggtccggcatgagaacagatgtgtggccctggaaaggtgtccctgcttccatcagggcatcgtacccgacacagagaccgacggagacggggggcccgtaccaggccgtactcttgtctacacaccgggacctttccacagggacgaaggtagtcccgtaggagtatgcccctggagaaacagtgaagattggctgcaacacttgtgtctgtcgggaccggaagtggaactgcacagaccatgtgtgtgatgccacgtgtcctcatacggggacctctttgtcacttctaaccgacgttgtgaacacagacagccctggccttcaccttgacgtgtctggtacacacactacggtgcacctccacgatcggcatggcccactacctcaccttcgacgggctcaaatacctgttccccggggagtgccagtacgttctggtgcaggattactgcggcagtgaggtgctagccgtaccgggtgatggagtggaagctgcccgagtttatggacaaggggcccctcacggtcatgcaagaccacgtcctaatgacgccgtcaaaccctgggacctttcggatcctagtggggaataagggatgcagccacccctcagtgaaatgcaagaaacgggtcaccatcctggtggagggaggagagattgggaccctggaaagcctaggatcaccccttattccctacgtcggtggggagtcactttacgttctttgcccagtggtaggaccacctccctcctctctttgagctgtttgacggggaggtgaatgtgaagaggcccatgaaggatgagactcactttgaggtggtggagtctggccggtacatcattctgctgctgggaactcgacaaactgcccctccacttacacttctccgggtacttcctactctgagtgaaactccaccacctcagaccggccatgtagtaagacgacgaccccaaagccctctccgtggtctgggaccgccacctgagcatctccgtggtcctgaagcagacataccaggagaaagtgtgtggcctgtgtgggaattttgatgtttcgggagaggcaccagaccctggcggtggactcgtagaggcaccaggacttcgtctgtatggtcctctttcacacaccggacacacccttaaaactaggcatccagaacaatgacctcaccagcagcaacctccaagtggaggaagaccctgtggactttgggaactcctggaaagtgagctcgcagtgtgctgacaccgtaggtcttgttactggagtggtcgtcgttggaggttcacctccttctgggacacctgaaacccttgaggacctttcactcgagcgtcacacgactgtccagaaaagtgcctctggactcatcccctgccacctgccataacaacatcatgaagcagacgatggtggattcctcctgtagaatccttaccagtgacgtggtcttttcacggagacctgagtaggggacggtggacggtattgttgtagtacttcgtctgctaccacctaaggaggacatcttaggaatggtcactgcacttccaggactgcaacaagctggtggaccccgagccatatctggatgtctgcatttacgacacctgctcctgtgagtccattggggactgcgcctgcttcgaaggtcctgacgttgttcgaccacctggggctcggtatagacctacagacgtaaatgctgtggacgaggacactcaggtaacccctgacgcggacgaagtgcgacaccattgctgcctatgcccacgtgtgtgcccagcatggcaaggtggtgacctggaggacggccacattgtgcccccagagctgcgaggagaggaacgctgtggtaacgacggatacgggtgcacacacgggtcgtaccgttccaccactggacctcctgccggtgtaacacgggggtctcgacgctcctctcctatctccgggagaacgggtatgagtgtgagtggcgctataacagctgtgcacctgcctgtcaagtcacgtgtcagcaccctgagccactggcctgccctgttagaggccctcttgcccatactcacactcaccgcgatattgtcgacacgtggacggacagttcagtgcacagtcgtgggactcggtgaccggacgggacagcagtgtgtggagggctgccatgcccactgccctccagggaaaatcctggatgagcttttgcagacctgcgttgaccctgaagactgtccagtgtgtgagcgtcacacacctcccgacggtacgggtgacgggaggtcccttttaggacctactcgaaaacgtctggacgcaactgggacttctgacaggtcacacactcgtggctggccggcgttttgcctcaggaaagaaagtcaccttgaatcccagtgaccctgagcactgccagatttgccactgtgatgttgtcaacctcacctcaccgaccggccgcaaaacggagtcctttctttcagtggaacttagggtcactgggactcgtgacggtctaaacggtgacactacaacagttggagtggagtgaagcctgccaggagccgggaggcctggtggtgcctcccacagatgccccggtgagccccaccactctgtatgtggaggacatctcggaaccgccgttcacttcggacggtcctcggccctccggaccaccacggagggtgtctacggggccactcggggtggtgagacatacacctcctgtagagccttggcggcaagcacgatttctactgcagcaggctactggacctggtcttcctgctggatggctcctccaggctgtccgaggctgagtttgaagtgctgaaggcctttgtgcgtgctaaagatgacgtcgtccgatgacctggaccagaaggacgacctaccgaggaggtccgacaggctccgactcaaacttcacgacttccggaaacacgtggacatgatggagcggctgcgcatctcccagaagtgggtccgcgtggccgtggtggagtaccacgacggctcccacgcctacatcgggctcaaggacccacctgtactacctcgccgacgcgtagagggtcttcacccaggcgcaccggcaccacctcatggtgctgccgagggtgcggatgtagcccgagttcctggggaagcgaccgtcagagctgcggcgcattgccagccaggtgaagtatgcgggcagccaggtggcctccaccagcgaggtcttgaaatacacactgttccaccttcgctggcagtctcgacgccgcgtaacggtcggtccacttcatacgcccgtcggtccaccggaggtggtcgctccagaactttatgtgtgacaaggtaatcttcagcaagatcgaccgccctgaagcctcccgcatcgccctgctcctgatggccagccaggagccccaacggatgtcccggaactttgtccgctacttagaagtcgttctagctggcgggacttcggagggcgtagcgggacgaggactaccggtcggtcctcggggttgcctacagggccttgaaacaggcgatggtccagggcctgaagaagaagaaggtcattgtgatcccggtgggcattgggccccatgccaacctcaagcagatccgcctcatcgagaagcaggcccctgcaggtcccggacttcttcttcttccagtaacactagggccacccgtaacccggggtacggttggagttcgtctaggcggagtagctcttcgtccggggacagaacaaggccttcgtgctgagcagtgtggatgagctggagcagcaaagggacgagatcgttagctacctctgtgaccttgcccctgaagcccctcctcctcttgttccggaagcacgactcgtcacacctactcgacctcgtcgtttccctgctctagcaatcgatggagacactggaacggggacttcggggaggaggtactctgccccccgacatggcacaagtcactgtgggcccggggctcttgggggtttcgaccctggggcccaagaggaactccatggttctggatgtggcgatgagacggggggctgtaccgtgttcagtgacacccgggccccgagaacccccaaagctgggaccccgggttctccttgaggtaccaagacctacaccgcttcgtcctggaaggatcggacaaaattggtgaagccgacttcaacaggagcaaggagttcatggaggaggtgattcagcggatggatgtgggccaggacaaagcaggaccttcctagcctgttttaaccacttcggctgaagttgtcctcgttcctcaagtacctcctccactaagtcgcctacctacacccggtcctgtgcatccacgtcacggtgctgcagtactcctacatggtgaccgtggagtaccccttcagcgaggcacagtccaaaggggacatcctgcagcgggtgcgagacgtaggtgcagtgccacgacgtcatgaggatgtaccactggcacctcatggggaagtcgctccgtgtcaggtttcccctgtaggacgtcgcccacgctctgatccgctaccagggcggcaacaggaccaacactgggctggccctgcggtacctctctgaccacagcttcttggtcagccagggtgaccgggagcaggcgctaggcgatggtcccgccgttgtcctggttgtgacccgaccgggacgccatggagagactggtgtcgaagaaccagtcggtcccactggccctcgtccgccccaacctggtctacatggtcaccggaaatcctgcctctgatgagatcaagaggctgcctggagacatccaggtggtgcccattggagtgggccctaatggggttggaccagatgtaccagtggcctttaggacggagactactctagttctccgacggacctctgtaggtccaccacgggtaacctcacccgggattacccaacgtgcaggagctggagaggattggctggcccaatgcccctatcctcatccaggactttgagacgctcccccgagaggctcctgacctggtgctgcaggttgcacgtcctcgacctctcctaaccgaccgggttacggggataggagtaggtcctgaaactctgcgagggggctctccgaggactggaccacgacgtgaggtgctgctccggagaggggctgcagatccccaccctctcccctgcacctgactgcagccagcccctggacgtgatccttctcctggatggctcctccctccacgacgaggcctctccccgacgtctaggggtgggagaggggacgtggactgacgtcggtcggggacctgcactaggaagaggacctaccgaggaggagtttcccagcttcttattttgatgaaatgaagagtttcgccaaggctttcatttcaaaagccaatatagggcctcgtctcactcaggtgtcagtgctgctcaaagggtcgaagaataaaactactttacttctcaaagcggttccgaaagtaaagttttcggttatatcccggagcagagtgagtccacagtcacgacgagtatggaagcatcaccaccattgacgtgccatggaacgtggtcccggagaaagcccatttgctgagccttgtggacgtcatgcagcgggagggaggccctcataccttcgtagtggtggtaactgcacggtaccttgcaccagggcctctttcgggtaaacgactcggaacacctgcagtacgtcgccctccctccgggcagccaaatcggggatgccttgggctttgctgtgcgatacttgacttcagaaatgcatggtgccaggccgggagcctcaaaggcggtggtcatcctggtcgtcggtttagcccctacggaacccgaaacgacacgctatgaactgaagtctttacgtaccacggtccggccctcggagtttccgccaccagtaggaccagacggacgtctctgtggattcagtggatgcagcagctgatgccgccaggtccaacagagtgacagtgttccctattggaattggagatcgctacgatgcagtgcctgcagagacacctaagtcacctacgtcgtcgactacggcggtccaggttgtctcactgtcacaagggataaccttaacctctagcgatgctacgtccccagctacggatcttggcaggcccagcaggcgactccaacgtggtgaagctccagcgaatcgaagacctccctaccatggtcaccttgggcaattccttgggtcgatgcctagaaccgtccgggtcgtccgctgaggttgcaccacttcgaggtcgcttagcttctggagggatggtaccagtggaacccgttaaggaacctccacaaactgtgctctggatttgttaggatttgcatggatgaggatgggaatgagaagaggcccggggacgtctggaccttgccagaccagtgccacggaggtgtttgacacgagacctaaacaatcctaaacgtacctactcctacccttactcttctccgggcccctgcagacctggaacggtctggtcacggtgaccgtgacttgccagccagatggccagaccttgctgaagagtcatcgggtcaactgtgaccgggggctgaggccttcgtgccctaacagccagtcccctgtggcactgaacggtcggtctaccggtctggaacgacttctcagtagcccagttgacactggcccccgactccggaagcacgggattgtcggtcaggggacttaaagtggaagagacctgtggctgccgctggacctgcccctgygtgtgcacaggcagctccactcggcacatcgtgacctttgatgggcagaatttcaaaatttcaccttctctggacaccgacggcgacctggacggggacrcacacgtgtccgtcgaggtgagccgtgtagcactggaaactacccgtcttaaagttgctgactggcagctgttcttatgtcctatttcaaaacaaggagcaggacctggaggtgattctccataatggtgcctgcagccctggagcaaggcagggccgactgaccgtcgacaagaatacaggataaagttttgttcctcgtcctggacctccactaagaggtattaccacggacgtcgggacctcgttccgtcccgtgcatgaaatccatcgaggtgaagcacagtgccctctccgtcgagstgcacagtgacatggaggtgacggtgaatgggagactggtctctgttccttacgacgtactttaggtagctccacttcgtgtcacgggagaggcagctcsacgtgtcactgtacctccactgccacttaccctctgaccagagacaaggaatgctgggtgggaacatggaagtcaacgtttatggtgccatcatgcatgaggtcagattcaatcaccttggtcacatcttcacattcactccacaaaacaatgaacccacccttgtaccttcagttgcaaataccacggtagtacgtactccagtctaagttagtggaaccagtgtagaagtgtaagtgaggtgttttgttactgttccaactgcagctcagccccaagacttttgcttcaaagacgtatggtctgtgtgggatctgtgatgagaacggagccaatgacttcatgctgagggatcaaggttgacgtcgagtcggggttctgaaaacgaagtttctgcataccagacacaccctagacactactcttgcctcggttactgaagtacgactccctaggcacagtcaccacagactggaaaacacttgttcaggaatggactgtgcagcggccagggcagacgtgccagcccatcctggaggagcagtgtcttgtccccgtgtcagtggtgtctgaccttttgtgaacaagtccttacctgacacgtcgccggtcccgtctgcacggtcgggtaggacctcctcgtcacagaacaggccgacagctcccactgccaggtcctcctcttaccactgtttgctgaatgccacaaggtcctggctccagccacattctatgccatctgccagcaggacagggctgtcgagggtgacggtccaggaggagaatggtgacaaacgacttacggtgttccaggaccgaggtcggtgtaagatacggtagacggtcgtcctgtcttgccaccaggagcaagtgtgtgaggtgatcgcctcttatgcccacctctgtcggaccaacggggtctgcgttgactggaggacacctgatttctgtgctaacggtggtcctcgttcacacactccactagcggagaatacgggtggagacagcctggttgccccagacgcaactgacctcctgtggactaaagacacgaatgtcatgcccaccatctctggtctacaaccactgtgagcatggctgtccccggcactgtgatggcaacgtgagctcctgtggggaccatccctccgaagtacagtacgggtggtagagaccagatgttggtgacactcgtaccgacaggggccgtgacactaccgttgcactcgaggacacccctggtagggaggcttcgctgtttctgccctccagataaagtcatgttggaaggcagctgtgtccctgaagaggcctgcactcagtgcattggtgaggatggagtccagcaccagttcgacaaagacgggaggtctatttcagtacaaccttccgtcgacacagggacttctccggacgtgagtcacgtaaccactcctacctcaggtcgtggtcaacctggaagcctgggtcccggaccaccagccctgtcagatctgcacatgcctcagcgggcggaaggtcaactgcacaacgcagccctgccccacggccaaaggaccttcggacccagggcctggtggtcgggacagtctagacgtgtacggagtcgcccgccttccagttgacgtgttgcgtcgggacggggtgccggtttgctcccacgtgtggcctgtgtgaagtagcccgcctccgccagaatgcagaccagtgctgccccgagtatgagtgtgtgtgtgacccagtgagctgtgacccgagggtgcacaccggacacacttcatcgggcggaggcggtcttacgtctggtcacgacggggctcatactcacacacacactgggtcactcgacactggtgcccccagtgcctcactgtgaacgtggcctccagcccacactgaccaaccctggcgagtgcagacccaacttcacctgcgcctgcaggaaggaggagtgacgggggtcacggagtgacacttgcaccggaggtcgggtgtgactggttgggaccgctcacgtctgggttgaagtggacgcggacgtccttcctcctcaccaaaagagtgtccccaccctcctgccccccgcaccgtttgcccacccttcggaagacccagtgctgtgatgagtatgagtgtgcctgcaactgtgtcaacgttttctcacaggggtgggaggacggggggcgtggcaaacgggtgggaagccttctgggtcacgacactactcatactcacacggacgttgacacagttgtccacagtgagctgtccccttgggtacttggcctcaaccgccaccaatgactgtggctgtaccacaaccacctgccttcccgacaaggtgtgtgtccaccaggtgtcactcgacaggggaacccatgaaccggagttggcggtggttactgacaccgacatggtgttggtggacggaagggctgttccacacacaggtgggaagcaccatctaccctgtgggccagttctgggaggagggctgcgatgtgtgcacctgcaccgacatggaggatgccgtgatgggcctccgcgtggcccacttcgtggtagatgggacacccggtcaagaccctcctcccgacgctacacacgtggacgtggctgtacctcctacggcactacccggaggcgcaccgggtgtgctcccagaagccctgtgaggacagctgtcggtcgggcttcacttacgttctgcatgaaggcgagtgctgtggaaggtgcctgccatctgcctgtgagcacgagggtcttcgggacactcctgtcgacagccagcccgaagtgaatgcaagacgtacttccgctcacgacaccttccacggacggtagacggacactcgtggtgactggctcaccgcggggggactcccagtcttcctggaagagtgtcggctcccagtgggcctccccggagaacccctgcctcatcaatgagtgtgcaccactgaccgagtggcgcccccctgagggtcagaaggaccttctcacagccgagggtcacccggaggggcctcttggggacggagtagttactcacactccgagtgaaggaggaggtctttatacaacaaaggaacgtctcctgcccccagctggaggtccctgtctgcccctcgggctttcagctgagctgtaagacaggctcacttcctcctccagaaatatgttgtttccttgcagaggacgggggtcgacctccagggacagacggggagcccgaaagtcgactcgacattctgctcagcgtgctgcccaagctgtcgctgtgagcgcatggaggcctgcatgctcaatggcactgtcattgggcccgggaagactgtgatgatcgatgtgtgcgagtcgcacgacgggttcgacagcgacactcgcgtacctccggacgtacgagttaccgtgacagtaacccgggcccttctgacactactagctacacacgacgacctgccgctgcatggtgcaggtgggggtcatctctggattcaagctggagtgcaggaagaccacctgcaacccctgccccctgggttacaaggaagtgctggacggcgacgtaccacgtccacccccagtagagacctaagttcgacctcacgtccttctggtggacgttggggacgggggacccaatgttccttcaaaataacacaggtgaatgttgtgggagatgtttgcctacggcttgcaccattcagctaagaggaggacagatcatgacactgaagcgtgatgagacgctttttattgtgtccacttacaacaccctctacaaacggatgccgaacgtggtaagtcgattctcctcctgtctagtactgtgacttcgcactactctgcgaccaggatggctgtgatactcacttctgcaaggtcaatgagagaggagagtacttctgggagaagagggtcacaggctgcccaccctttgatgaacacaagggtcctaccgacactatgagtgaagacgttccagttactctctcctctcatgaagaccctcttctcccagtgtccgacgggtgggaaactacttgtgttctgtcttgctgagggaggtaaaattatgaaaattccaggcacctgctgtgacacatgtgaggagcctgagtgcaacgacatcactgccaggctgcagtatgacagaacgactccctccattttaatacttttaaggtccgtggacgacactgtgtacactcctcggactcacgttgctgtagtgacggtccgacgtcatactcaaggtgggaagctgtaagtctgaagtagaggtggatatccactactgccagggcaaatgtgccagcaaagccatgtactccattgacatcaacgatgtagttccacccttcgacattcagacttcatctccacctataggtgatgacggtcccgtttacacggtcgtttcggtacatgaggtaactgtagttgctacagcaggaccagtgctcctgctgctctccgacacggacggagcccatgcaggtggccctgcactgcaccaatggctctgttgtgtaccatgaggttctcaatcgtcctggtcacgaggacgacgagaggctgtgcctgcctcgggtacgtccaccgggacgtgacgtggttaccgagacaacacatggtactccaagagttagccatggagtgcaaatgctcccccaggaagtgcagcaagtga

SEQ ID NO: 2 - protein, 2813 aa, Homo sapiens
  misc_feature (1)..(22): VWF Signal Peptide
  misc_feature (23)..(763): VWF D1D2 region
  misc_feature (764)..(866): VWF D'Domain
  misc_feature (867)..(1240): VWF D3 Domain
  misc_feature (1241)..(1479): VWF A1 Domain
  variant (2016)..(2016): Xaa can be any naturally occurring amino acid
MIPARFAGVLLALALILPGTLCAEGTRGRSSTARCSLFGSDFVNTFDGSMYSFAGYCSYLLAGGCQKRSFSIIGDFQNGKRVSLSVYLGEFFDIHLFVNGTVTQGDQRVSMPYASKGLYLETEAGYYKLSGEAYGFVARIDGSGNFQVLLSDRYFNKTCGLCGNFNIFAEDDFMTQEGTLTSDPYDFANSWALSSGEQWCERASPPSSSCNISSGEMQKGLWEQCQLLKSTSVFARCHPLVDPEPFVALCEKTLCECAGGLECACPALLEYARTCAQEGMVLYGWTDHSACSPVCPAGMEYRQCVSPCARTCQSLHINEMCQERCVDGCSCPEGQLLDEGLCVESTECPCVHSGKRYPPGTSLSRDCNTCICRNSQWICSNEECPGECLVTGQSHFKSFDNRYFTFSGICQYLLARDCQDHSFSIVIETVQCADDRDAVCTRSVTVRLPGLHNSLVKLKHGAGVAMDGQDIQLPLLKGDLRIQHTVTASVRLSYGEDLQMDWDGRGRLLVKLSPVYAGKTCGLCGNYNGNQGDDFLTPSGLAEPRVEDFGNAWKLHGDCQDLQKQHSDPCALNPRMTRFSEEACAVLTSPTFEACHRAVSPLPYLRNCRYDVCSCSDGRECLCGALASYAAACAGRGVRVAWREPGRCELNCPKGQVYLQCGTPCNLTCRSLSYPDEECNEACLEGCFCPPGLYMDERGDCVPKAQCPCYYDGEIFQPEDIFSDHHTMCYCEDGFMHCTMSGVPGSLLPDAVLSSPLSHRSKRSLSCRPPMVKLVCPADNLRAEGLECTKTCQNYDLECMSMGCVSGCLCPPGMVRHENRCVALERCPCFHQGKEYAPGETVKIGCNTCVCRDRKWNCTDHVCDATCSTIGMAHYLTFDGLKYLFPGECQYVLVQDYCGSNPGTFRILVGNKGCSHPSVKCKKRVTILVEGGEIELFDGEVNVKRPMKDETHFEVVESGRYIILLLGKALSVVWDRHLSISVVLKQTYQEKVCGLCGNFDGIQNNDLTSSNLQVEEDPVDFGNSWKVSSQCADTRKVPLDSSPATCHNNIMKQTMVDSSCRILTSDVFQDCNKLVDPEPYLDVCIYDTCSCESIGDCACFCDTIAAYAHVCAQHGKVVTWRTATLCPQSCEERNLRENGYECEWRYNSCAPACQVTCQHPEPLACPVQCVEGCHAHCPPGKILDELLQTCVDPEDCPVCEVAGRRFASGKKVTLNPSDPEHCQICHCDVVNLTCEACQEPGGLVVPPTDAPVSPTTLYVEDISEPPLHDFYCSRLLDLVFLLDGSSRLSEAEFEVLKAFVVDMMERLRISQKWVRVAVVEYHDGSHAYIGLKDRKRPSELRRIASQVKYAGSQVASTSEVLKYTLFQIFSKIDRPEASRIALLLMASQEPQRMSRNFVRYVQGLKKKKVIVIPVGIGPHANLKQIRLIEKQAPENKAFVLSSVDELEQQRDEIVSYLCDLAPEAPPPTLPPDMAQVTVGPGLLGVSTLGPKRNSMVLDVAFVLEGSDKIGEADFNRSKEFMEEVIQRMDVGQDSIHVTVLQYSYMVTVEYPFSEAQSKGDILQRVREIRYQGGNRTNTGLALRYLSDHSFLVSQGDREQAPNLVYMVTGNPASDEIKRLPGDIQVVPIGVGPNANVQELERIGWPNAPILIQDFETLPREAPDLVLQRCCSGEGLQIPTLSPAPDCSQPLDVILLLDGSSSFPASYFDEMKSFAKAFISKANIGPRLTQVSVLQYGSITTIDVPWNVVPEKAHLLSLVDVMQREGGPSQIGDALGFAVRYLTSEMHGARPGASKAVVILVTDVSVDSVDAAADAARSNRVTVFPIGIGDRYDAAQLRILAGPAGDSNVVKLQRIEDLPTMVTLGNSFLHKLCSGFVRICMDEDGNEKRPGDVWTLPDQCHTVTCQPDGQTLLKSHRVNCDRGLRPSCPNSQSPVKVEETCGCRWTCPCVCTGSSTRHIVTFDGQNFKLTGSCSYVLFQNKEQDLEVILHNGACSPGARQGCMKSIEVKHSALSVEXHSDMEVTVNGRLVSVPYVGGNMEVNVYGAIMHEVRFNHLGHIFTFTPQNNEFQLQLSPKTFASKTYGLCGICDENGANDFMLRDGTVTTDWKTLVQEWTVQRPGQTCQPILEEQCLVPDSSHCQVLLLPLFAECHKVLAPATFYAICQQDSCHQEQVCEVIASYAHLCRTNGVCVDWRTPDFCAMSCPPSLVYNHCEHGCPRHCDGNVSSCGDHPSEGCFCPPDKVMLEGSCVPEEACTQCIGEDGVQHQFLEAWVPDHQPCQICTCLSGRKVNCTTQPCPTAKAPTCGLCEVARLRQNADQCCPEYECVCDPVSCDLPPVPHCERGLQPTLTNPGECRPNFTCACRKEECKRVSPPSCPPHRLPTLRKTQCCDEYECACNCVNSTVSCPLGYLASTATNDCGCTTTTCLPDKVCVHRSTIYPVGQFWEEGCDVCTCTDMEDAVMGLRVAQCSQKPCEDSCRSGFTYVLHEGECCGRCLPSACEVVTGSPRGDSQSSWKSVGSQWASPENPCLINECVRVKEEVFIQQRNVSCPQLEVPVCPSGFQLSCKTSACCPSCRCERMEACMLNGTVIGPGKTVMIDVCTTCRCMVQVGVISGFKLECRKTTCNPCPLGYKEENNTGECCGRCLPTACTIQLRGGQIMTLKRDETLQDGCDTHFCKVNERGEYFWEKRVTGCPPFDEHKCLAEGGKIMKIPGTCCDTCEEPECNDITARLQYVKVGSCKSEVEVDIHYCQGKCASKAMYSIDINDVQDQCSCCSPTRTEPMQVALHCTNGSVVYHEVLNAMECKCSPRKCSK

SEQ ID NO: 3 - protein, 11 aa, Artificial Sequence
  polypeptide
PKNSSMISNTP

SEQ ID NO: 4 - protein, 7 aa, Artificial
  polypeptide
HQSLGTQ

SEQ ID NO: 5 - protein, 8 aa, Artificial
  polypeptide
HQNLSDGK

SEQ ID NO: 6 - protein, 8 aa, Artificial
  polypeptide
HQNISDGK

SEQ ID NO: 7 - protein, 8 aa, Artificial
  polypeptide
VISSHLGQ

SEQ ID NO: 8 - protein, 20 aa, Artificial
  PAS sequence
ASPAAPAPASPAAPAPSAPA

SEQ ID NO: 9 - protein, 20 aa, Artificial
  PAS sequence
AAPASPAPAAPSAPAPAAPS

SEQ ID NO: 10 - protein, 20 aa, Artificial
  PAS sequence
APSSPSPSAPSSPSPASPSS

SEQ ID NO: 11 - protein, 19 aa, Artificial
  PAS sequence
APSSPSPSAPSSPSPASPS

SEQ ID NO: 12 - protein, 20 aa, Artificial
  PAS sequence
SSPSAPSPSSPASPSPSSPA

SEQ ID NO: 13 - protein, 24 aa, Artificial
  PAS sequence
AASPAAPSAPPAAASPAAPSAPPA

SEQ ID NO: 14 - protein, 20 aa, Artificial
  PAS sequence
ASAAAPAAASAAASAPSAAA

SEQ ID NO: 15 - protein, 19 aa, Artificial
  FVIII signal peptide
MQIELSTCFFLCLLRFCFS

SEQ ID NO: 16 - protein, 2332 aa, Homo sapiens
ATRRYYLGAVELSWDYMQSDLGELPVDARFPPRVPKSFPFNTSVVYKKTLFVEFTDHLFNIAKPRPPWMGLLGPTIQAEVYDTVVITLKNMASHPVSLHAVGVSYWKASEGAEYDDQTSQREKEDDKVFPGGSHTYVWQVLKENGPMASDPLCLTYSYLSHVDLVKDLNSGLIGALLVCREGSLAKEKTQTLHKFILLFAVFDEGKSWHSETKNSLMQDRDAASARAWPKMHTVNGYVNRSLPGLIGCHRKSVYWHVIGMGTTPEVHSIFLEGHTFLVRNHRQASLEISPITFLTAQTLLMDLGQFLLFCHISSHQHDGMEAYVKVDSCPEEPQLRMKNNEEAEDYDDDLTDSEMDVVRFDDDNSPSFIQIRSVAKKHPKTWVHYIAAEEEDWDYAPLVLAPDDRSYKSQYLNNGPQRIGRKYKKVRFMAYTDETFKTREAIQHESGILGPLLYGEVGDTLLIIFKNQASRPYNIYPHGITDVRPLYSRRLPKGVKHLKDFPILPGEIFKYKWTVTVEDGPTKSDPRCLTRYYSSFVNMERDLASGLIGPLLICYKESVDQRGNQIMSDKRNVILFSVFDENRSWYLTENIQRFLPNPAGVQLEDPEFQASNIMHSINGYVFDSLQLSVCLHEVAYWYILSIGAQTDFLSVFFSGYTFKHKMVYEDTLTLFPFSGETVFMSMENPGLWILGCHNSDFRNRGMTALLKVSSCDKNTGDYYEDSYEDISAYLLSKNNAIEPRSFSQNSRHPSTRQKQFNATTIPENDIEKTDPWFAHRTPMPKIQNVSSSDLLMLLRQSPTPHGLSLSDLQEAKYETFSDDPSPGAIDSNNSLSEMTHFRPQLHHSGDMVFTPESGLQLRLNEKLGTTAATELKKLDFKVSSTSNNLISTIPSDNLAAGTDNTSSLGPPSMPVHYDSQLDTTLFGKKSSPLTESGGPLSLSEENNDSKLLESGLMNSQESSWGKNVSSTESGRLFKGKRAHGPALLTKDNALFKVSISLLKTNKTSNNSATNRKTHIDGPSLLIENSPSVWQNILESDTEFKKVTPLIHDRMLMDKNATALRLNHMSNKTTSSKNMEMVQQKKEGPIPPDAQNPDMSFFKMLFLPESARWIQRTHGKNSLNSGQGPSPKQLVSLGPEKSVEGQNFLSEKNKVVVGKGEFTKDVGLKEMVFPSSRNLFLTNLDNLHENNTHNQEKKIQEEIEKKETLIQENVVLPQIHTVTGTKNFMKNLFLLSTRQNVEGSYDGAYAPVLQDFRSLNDSTNRTKKHTAHFSKKGEEENLEGLGNQTKQIVEKYACTTRISPNTSQQNFVTQRSKRALKQFRLPLEETELEKRIIVDDTSTQWSKNMKHLTPSTLTQIDYNEKEKGAITQSPLSDCLTRSHSIPQANRSPLPIAKVSSFPSIRPIYLTRVLFQDNSSHLPAASYRKKDSGVQESSHFLQGAKKNNLSLAILTLEMTGDQREVGSLGTSATNSVTYKKVENTVLPKPDLPKTSGKVELLPKVHIYQKDLFPTETSNGSPGHLDLVEGSLLQGTEGAIKWNEANRPGKVPFLRVATESSAKTPSKLLDPLAWDNHYGTQIPKEEWKSQEKSPEKTAFKKKDTILSLNACESNHAIAAINEGQNKPEIEVTWAKQGRTERLCSQNPPVLKRHQREITRTTLQSDQEEIDYDDTISVEMKKEDFDIYDEDENQSPRSFQKKTRHYFIAAVERLWDYGMSSSPHVLRNRAQSGSVPQFKKVVFQEFTDGSFTQPLYRGELNEHLGLLGPYIRAEVEDNIMVTFRNQASRPYSFYSSLISYEEDQRQGAEPRKNFVKPNETKTYFWKVQHHMAPTKDEFDCKAWAYFSDVDLEKDVHSGLIGPLLVCHTNTLNPAHGRQVTVQEFALFFTIFDETKSWYFTENMERNCRAPCNIQMEDPTFKENYRFHAINGYIMDTLPGLVMAQDQRIRWYLLSMGSNENIHSIHFSGHVFTVRKKEEYKMALYNLYPGVFETVEMLPSKAGIWRVECLIGEHLHAGMSTLFLVYSNKCQTPLGMASGHIRDFQITASGQYGQWAPKLARLHYSGSINAWSTKEPFSWIKVDLLAPMIIHGIKTQGARQKFSSLYISQFIIMYSLDGKKWQTYRGNSTGTLMVFFGNVDSSGIKHNIFNPPIIARYIRLHPTHYSIRSTLRMELMGCDLNSCSMPLGMESKAISDAQITASSYFTNMFATWSPSKARLHLQGRSNAWRPQVNNPKEWLQVDFQKTMKVTGVTTQGVKSLLTSMYVKEFLISSSQDGHQWTLFFQNGKVKVFQGNQDSFTPVVNSLDPPLLTRYLRIHPQSWVHQIALRMEVLGCEAQDLY

SEQ ID NO: 17 - DNA, 7053 bp, Homo sapiens
atgcaaatagagctctccacctgcttctttctgtgccttttgcgattctgctttagtgccaccagaagatactacctgggtgcagtggaactgtcatgggactatatgcaaagtgatctcggtgagctgcctgtggacgcaagatttcctcctagagtgccaaaatcttttccattcaacacctcagtcgtgtacaaaaagactctgtttgtagaattcacggatcaccttttcaacatcgctaagccaaggccaccctggatgggtctgctaggtcctaccatccaggctgaggtttatgatacagtggtcattacacttaagaacatggcttcccatcctgtcagtcttcatgctgttggtgtatcctactggaaagcttctgagggagctgaatatgatgatcagaccagtcaaagggagaaagaagatgataaagtcttccctggtggaagccatacatatgtctggcaggtcctgaaagagaatggtccaatggcctctgacccactgtgccttacctactcatatctttctcatgtggacctggtaaaagacttgaattcaggcctcattggagccctactagtatgtagagaagggagtctggccaaggaaaagacacagaccttgcacaaatttatactactttttgctgtatttgatgaagggaaaagttggcactcagaaacaaagaactccttgatgcaggatagggatgctgcatctgctcgggcctggcctaaaatgcacacagtcaatggttatgtaaacaggtctctgccaggtctgattggatgccacaggaaatcagtctattggcatgtgattggaatgggcaccactcctgaagtgcactcaatattcctcgaaggtcacacatttcttgtgaggaaccatcgccaggcgtccttggaaatctcgccaataactttccttactgctcaaacactcttgatggaccttggacagtttctactgttttgtcatatctcttcccaccaacatgatggcatggaagcttatgtcaaagtagacagctgtccagaggaaccccaactacgaatgaaaaataatgaagaagcggaagactatgatgatgatcttactgattctgaaatggatgtggtcaggtttgatgatgacaactctccttcctttatccaaattcgctcagttgccaagaagcatcctaaaacttgggtacattacattgctgctgaagaggaggactgggactatgctcccttagtcctcgcccccgatgacagaagttataaaagtcaatatttgaacaatggccctcagcggattggtaggaagtacaaaaaagtccgatttatggcatacacagatgaaacctttaagactcgtgaagctattcagcatgaatcaggaatcttgggacctttactttatggggaagttggagacacactgttgattatatttaagaatcaagcaagcagaccatataacatctaccctcacggaatcactgatgtccgtcctttgtattcaaggagattaccaaaaggtgtaaaacatttgaaggattttccaattctgccaggagaaatattcaaatataaatggacagtgactgtagaagatgggccaactaaatcagatcctcggtgcctgacccgctattactctagtttcgttaatatggagagagatctagcttcaggactcattggccctctcctcatctgctacaaagaatctgtagatcaaagaggaaaccagataatgtcagacaagaggaatgtcatcctgttttctgtatttgatgagaaccgaagctggtacctcacagagaatatacaacgctttctccccaatccagctggagtgcagcttgaggatccagagttccaagcctccaacatcatgcacagcatcaatggctatgtttttgatagtttgcagttgtcagtttgtttgcatgaggtggcatactggtacattctaagcattggagcacagactgacttcctttctgtcttcttctctggatataccttcaaacacaaaatggtctatgaagacacactcaccctattcccattctcaggagaaactgtcttcatgtcgatggaaaacccaggtctatggattctggggtgccacaactcagactttcggaacagaggcatgaccgccttactgaaggtttctagttgtgacaagaacactggtgattattacgaggacagttatgaagatatttcagcatacttgctgagtaaaaacaatgccattgaaccaagaagcttctcccagaattcaagacaccctagcactaggcaaaagcaatttaatgccaccacaattccagaaaatgacatagagaagactgacccttggtttgcacacagaacacctatgcctaaaatacaaaatgtctcctctagtgatttgttgatgctcttgcgacagagtcctactccacatgggctatccttatctgatctccaagaagccaaatatgagactttttctgatgatccatcacctggagcaatagacagtaataacagcctgtctgaaatgacacacttcaggccacagctccatcacagtggggacatggtatttacccctgagtcaggcctccaattaagattaaatgagaaactggggacaactgcagcaacagagttgaagaaacttgatttcaaagtttctagtacatcaaataatctgatttcaacaattccatcagacaatttggcagcaggtactgataatacaagttccttaggacccccaagtatgccagttcattatgatagtcaattagataccactctatttggcaaaaagtcatctccccttactgagtctggtggacctctgagcttgagtgaagaaaataatgattcaaagttgttagaatcaggtttaatgaatagccaagaaagttcatggggaaaaaatgtatcgtcaacagagagtggtaggttatttaaagggaaaagagctcatggacctgctttgttgactaaagataatgccttattcaaagttagcatctctttgttaaagacaaacaaaacttccaataattcagcaactaatagaaagactcacattgatggcccatcattattaattgagaatagtccatcagtctggcaaaatatattagaaagtgacactgagtttaaaaaagtgacacctttgattcatgacagaatgcttatggacaaaaatgctacagctttgaggctaaatcatatgtcaaataaaactacttcatcaaaaaacatggaaatggtccaacagaaaaaagagggccccattccaccagatgcacaaaatccagatatgtcgttctttaagatgctattcttgccagaatcagcaaggtggatacaaaggactcatggaaagaactctctgaactctgggcaaggccccagtccaaagcaattagtatccttaggaccagaaaaatctgtggaaggtcagaatttcttgtctgagaaaaacaaagtggtagtaggaaagggtgaatttacaaaggacgtaggactcaaagagatggtttttccaagcagcagaaacctatttcttactaacttggataatttacatgaaaataatacacacaatcaagaaaaaaaaattcaggaagaaatagaaaagaaggaaacattaatccaagagaatgtagttttgcctcagatacatacagtgactggcactaagaatttcatgaagaaccttttcttactgagcactaggcaaaatgtagaaggttcatatgacggggcatatgctccagtacttcaagattttaggtcattaaatgattcaacaaatagaacaaagaaacacacagctcatttctcaaaaaaaggggaggaagaaaacttggaaggcttgggaaatcaaaccaagcaaattgtagagaaatatgcatgcaccacaaggatatctcctaatacaagccagcagaattttgtcacgcaacgtagtaagagagctttgaaacaattcagactcccactagaagaaacagaacttgaaaaaaggataattgtggatgacacctcaacccagtggtccaaaaacatgaaacatttgaccccgagcaccctcacacagatagactacaatgagaaggagaaaggggccattactcagtctcccttatcagattgccttacgaggagtcatagcatccctcaagcaaatagatctccattacccattgcaaaggtatcatcatttccatctattagacctatatatctgaccagggtcctattccaagacaactcttctcatcttccagcagcatcttatagaaagaaagattctggggtccaagaaagcagtcatttcttacaaggagccaaaaaaaataacctttctttagccattctaaccttggagatgactggtgatcaaagagaggttggctccctggggacaagtgccacaaattcagtcacatacaagaaagttgagaacactgttctcccgaaaccagacttgcccaaaacatctggcaaagttgaattgcttccaaaagttcacatttatcagaaggacctattccctacggaaactagcaatgggtctcctggccatctggatctcgtggaagggagccttcttcagggaacagagggagcgattaagtggaatgaagcaaacagacctggaaaagttccctttctgagagtagcaacagaaagctctgcaaagactccctccaagctattggatcctcttgcttgggataaccactatggtactcagataccaaaagaagagtggaaatcccaagagaagtcaccagaaaaaacagcttttaagaaaaaggataccattttgtccctgaacgcttgtgaaagcaatcatgcaatagcagcaataaatgagggacaaaataagcccgaaatagaagtcacctgggcaaagcaaggtaggactgaaaggctgtgctctcaaaacccaccagtcttgaaacgccatcaacgggaaataactcgtactactcttcagtcagatcaagaggaaattgactatgatgataccatatcagttgaaatgaagaaggaagattttgacatttatgatgaggatgaaaatcagagcccccgcagctttcaaaagaaaacacgacactattttattgctgcagtggagaggctctgggattatgggatgagtagctccccacatgttctaagaaacagggctcagagtggcagtgtccctcagttcaagaaagttgttttccaggaatttactgatggctcctttactcagcccttataccgtggagaactaaatgaacatttgggactcctggggccatatataagagcagaagttgaagataatatcatggtaactttcagaaatcaggcctctcgtccctattccttctattctagccttatttcttatgaggaagatcagaggcaaggagcagaacctagaaaaaactttgtcaagcctaatgaaaccaaaacttacttttggaaagtgcaacatcatatggcacccactaaagatgagtttgactgcaaagcctgggcttatttctctgatgttgacctggaaaaagatgtgcactcaggcctgattggaccccttctggtctgccacactaacacactgaaccctgctcatgggagacaagtgacagtacaggaatttgctctgtttttcaccatctttgatgagaccaaaagctggtacttcactgaaaatatggaaagaaactgcagggctccctgcaatatccagatggaagatcccacttttaaagagaattatcgcttccatgcaatcaatggctacataatggatacactacctggcttagtaatggctcaggatcaaaggattcgatggtatctgctcagcatgggcagcaatgaaaacatccattctattcatttcagtggacatgtgttcactgtacgaaaaaaagaggagtataaaatggcactgtacaatctctatccaggtgtttttgagacagtggaaatgttaccatccaaagctggaatttggcgggtggaatgccttattggcgagcatctacatgctgggatgagcacactttttctggtgtacagcaataagtgtcagactcccctgggaatggcttctggacacattagagattttcagattacagcttcaggacaatatggacagtgggccccaaagctggccagacttcattattccggatcaatcaatgcctggagcaccaaggagcccttttcttggatcaaggtggatctgttggcaccaatgattattcacggcatcaagacccagggtgcccgtcagaagttctccagcctctacatctctcagtttatcatcatgtatagtcttgatgggaagaagtggcagacttatcgaggaaattccactggaaccttaatggtcttctttggcaatgtggattcatctgggataaaacacaatatttttaaccctccaattattgctcgatacatccgtttgcacccaactcattatagcattcgcagcactcttcgcatggagttgatgggctgtgatttaaatagttgcagcatgccattgggaatggagagtaaagcaatatcagatgcacagattactgcttcatcctactttaccaatatgtttgccacctggtctccttcaaaagctcgacttcacctccaagggaggagtaatgcctggagacctcaggtgaataatccaaaagagtggctgcaagtggacttccagaagacaatgaaagtcacaggagtaactactcagggagtaaaatctctgcttaccagcatgtatgtgaaggagttcctcatctccagcagtcaagatggccatcagtggactctcttttttcagaatggcaaagtaaaggtttttcagggaaatcaagactccttcacacctgtggtgaactctctagacccaccgttactgactcgctaccttcgaattcacccccagagttgggtgcaccagattgccctgaggatggaggttctgggctgcgaggcacaggacctctac

SEQ ID NO: 18 - protein, 1438 aa, Artificial
  BDD FVIII
ATRRYYLGAVELSWDYMQSDLGELPVDARFPPRVPKSFPFNTSVVYKKTLFVEFTDHLFNIAKPRPPWMGLLGPTIQAEVYDTVVITLKNMASHPVSLHAVGVSYWKASEGAEYDDQTSQREKEDDKVFPGGSHTYVWQVLKENGPMASDPLCLTYSYLSHVDLVKDLNSGLIGALLVCREGSLAKEKTQTLHKFILLFAVFDEGKSWHSETKNSLMQDRDAASARAWPKMHTVNGYVNRSLPGLIGCHRKSVYWHVIGMGTTPEVHSIFLEGHTFLVRNHRQASLEISPITFLTAQTLLMDLGQFLLFCHISSHQHDGMEAYVKVDSCPEEPQLRMKNNEEAEDYDDDLTDSEMDVVRFDDDNSPSFIQIRSVAKKHPKTWVHYIAAEEEDWDYAPLVLAPDDRSYKSQYLNNGPQRIGRKYKKVRFMAYTDETFKTREAIQHESGILGPLLYGEVGDTLLIIFKNQASRPYNIYPHGITDVRPLYSRRLPKGVKHLKDFPILPGEIFKYKWTVTVEDGPTKSDPRCLTRYYSSFVNMERDLASGLIGPLLICYKESVDQRGNQIMSDKRNVILFSVFDENRSWYLTENIQRFLPNPAGVQLEDPEFQASNIMHSINGYVFDSLQLSVCLHEVAYWYILSIGAQTDFLSVFFSGYTFKHKMVYEDTLTLFPFSGETVFMSMENPGLWILGCHNSDFRNRGMTALLKVSSCDKNTGDYYEDSYEDISAYLLSKNNAIEPRSFSQNPPVLKRHQREITRTTLQSDQEEIDYDDTISVEMKKEDFDIYDEDENQSPRSFQKKTRHYFIAAVERLWDYGMSSSPHVLRNRAQSGSVPQFKKVVFQEFTDGSFTQPLYRGELNEHLGLLGPYIRAEVEDNIMVTFRNQASRPYSFYSSLISYEEDQRQGAEPRKNFVKPNETKTYFWKVQHHMAPTKDEFDCKAWAYFSDVDLEKDVHSGLIGPLLVCHTNTLNPAHGRQVTVQEFALFFTIFDETKSWYFTENMERNCRAPCNIQMEDPTFKENYRFHAINGYIMDTLPGLVMAQDQRIRWYLLSMGSNENIHSIHFSGHVFTVRKKEEYKMALYNLYPGVFETVEMLPSKAGIWRVECLIGEHLHAGMSTLFLVYSNKCQTPLGMASGHIRDFQITASGQYGQWAPKLARLHYSGSINAWSTKEPFSWIKVDLLAPMIIHGIKTQGARQKFSSLYISQFIIMYSLDGKKWQTYRGNSTGTLMVFFGNVDSSGIKHNIFNPPIIARYIRLHPTHYSIRSTLRMELMGCDLNSCSMPLGMESKAISDAQITASSYFTNMFATWSPSKARLHLQGRSNAWRPQVNNPKEWLQVDFQKTMKVTGVTTQGVKSLLTSMYVKEFLISSSQDGHQWTLFFQNGKVKVFQGNQDSFTPVVNSLDPPLLTRYLRIHPQSWVHQIALRMEVLGCEAQDLY

SEQ ID NO: 19 - DNA, 4371 bp, Artificial
  BDD FVIII
atgcaaatagagctctccacctgcttctttctgtgccttttgcgattctgctttagtgccaccagaagatactacctgggtgcagtggaactgtcatgggactatatgcaaagtgatctcggtgagctgcctgtggacgcaagatttcctcctagagtgccaaaatcttttccattcaacacctcagtcgtgtacaaaaagactctgtttgtagaattcacggatcaccttttcaacatcgctaagccaaggccaccctggatgggtctgctaggtcctaccatccaggctgaggtttatgatacagtggtcattacacttaagaacatggcttcccatcctgtcagtcttcatgctgttggtgtatcctactggaaagcttctgagggagctgaatatgatgatcagaccagtcaaagggagaaagaagatgataaagtcttccctggtggaagccatacatatgtctggcaggtcctgaaagagaatggtccaatggcctctgacccactgtgccttacctactcatatctttctcatgtggacctggtaaaagacttgaattcaggcctcattggagccctactagtatgtagagaagggagtctggccaaggaaaagacacagaccttgcacaaatttatactactttttgctgtatttgatgaagggaaaagttggcactcagaaacaaagaactccttgatgcaggatagggatgctgcatctgctcgggcctggcctaaaatgcacacagtcaatggttatgtaaacaggtctctgccaggtctgattggatgccacaggaaatcagtctattggcatgtgattggaatgggcaccactcctgaagtgcactcaatattcctcgaaggtcacacatttcttgtgaggaaccatcgccaggcgtccttggaaatctcgccaataactttccttactgctcaaacactcttgatggaccttggacagtttctactgttttgtcatatctcttcccaccaacatgatggcatggaagcttatgtcaaagtagacagctgtccagaggaaccccaactacgaatgaaaaataatgaagaagcggaagactatgatgatgatcttactgattctgaaatggatgtggtcaggtttgatgatgacaactctccttcctttatccaaattcgctcagttgccaagaagcatcctaaaacttgggtacattacattgctgctgaagaggaggactgggactatgctcccttagtcctcgcccccgatgacagaagttataaaagtcaatatttgaacaatggccctcagcggattggtaggaagtacaaaaaagtccgatttatggcatacacagatgaaacctttaagactcgtgaagctattcagcatgaatcaggaatcttgggacctttactttatggggaagttggagacacactgttgattatatttaagaatcaagcaagcagaccatataacatctaccctcacggaatcactgatgtccgtcctttgtattcaaggagattaccaaaaggtgtaaaacatttgaaggattttccaattctgccaggagaaatattcaaatataaatggacagtgactgtagaagatgggccaactaaatcagatcctcggtgcctgacccgctattactctagtttcgttaatatggagagagatctagcttcaggactcattggccctctcctcatctgctacaaagaatctgtagatcaaagaggaaaccagataatgtcagacaagaggaatgtcatcctgttttctgtatttgatgagaaccgaagctggtacctcacagagaatatacaacgctttctccccaatccagctggagtgcagcttgaggatccagagttccaagcctccaacatcatgcacagcatcaatggctatgtttttgatagtttgcagttgtcagtttgtttgcatgaggtggcatactggtacattctaagcattggagcacagactgacttcctttctgtcttcttctctggatataccttcaaacacaaaatggtctatgaagacacactcaccctattcccattctcaggagaaactgtcttcatgtcgatggaaaacccaggtctatggattctggggtgccacaactcagactttcggaacagaggcatgaccgccttactgaaggtttctagttgtgacaagaacactggtgattattacgaggacagttatgaagatatttcagcatacttgctgagtaaaaacaatgccattgaaccaagaagcttctctcaaaacccaccagtcttgaaacgccatcaacgggaaataactcgtactactcttcagtcagatcaagaggaaattgactatgatgataccatatcagttgaaatgaagaaggaagattttgacatttatgatgaggatgaaaatcagagcccccgcagctttcaaaagaaaacacgacactattttattgctgcagtggagaggctctgggattatgggatgagtagctccccacatgttctaagaaacagggctcagagtggcagtgtccctcagttcaagaaagttgttttccaggaatttactgatggctcctttactcagcccttataccgtggagaactaaatgaacatttgggactcctggggccatatataagagcagaagttgaagataatatcatggtaactttcagaaatcaggcctctcgtccctattccttctattctagccttatttcttatgaggaagatcagaggcaaggagcagaacctagaaaaaactttgtcaagcctaatgaaaccaaaacttacttttggaaagtgcaacatcatatggcacccactaaagatgagtttgactgcaaagcctgggcttatttctctgatgttgacctggaaaaagatgtgcactcaggcctgattggaccccttctggtctgccacactaacacactgaaccctgctcatgggagacaagtgacagtacaggaatttgctctgtttttcaccatctttgatgagaccaaaagctggtacttcactgaaaatatggaaagaaactgcagggctccctgcaatatccagatggaagatcccacttttaaagagaattatcgcttccatgcaatcaatggctacataatggatacactacctggcttagtaatggctcaggatcaaaggattcgatggtatctgctcagcatgggcagcaatgaaaacatccattctattcatttcagtggacatgtgttcactgtacgaaaaaaagaggagtataaaatggcactgtacaatctctatccaggtgtttttgagacagtggaaatgttaccatccaaagctggaatttggcgggtggaatgccttattggcgagcatctacatgctgggatgagcacactttttctggtgtacagcaataagtgtcagactcccctgggaatggcttctggacacattagagattttcagattacagcttcaggacaatatggacagtgggccccaaagctggccagacttcattattccggatcaatcaatgcctggagcaccaaggagcccttttcttggatcaaggtggatctgttggcaccaatgattattcacggcatcaagacccagggtgcccgtcagaagttctccagcctctacatctctcagtttatcatcatgtatagtcttgatgggaagaagtggcagacttatcgaggaaattccactggaaccttaatggtcttctttggcaatgtggattcatctgggataaaacacaatatttttaaccctccaattattgctcgatacatccgtttgcacccaactcattatagcattcgcagcactcttcgcatggagttgatgggctgtgatttaaatagttgcagcatgccattgggaatggagagtaaagcaatatcagatgcacagattactgcttcatcctactttaccaatatgtttgccacctggtctccttcaaaagctcgacttcacctccaagggaggagtaatgcctggagacctcaggtgaataatccaaaagagtggctgcaagtggacttccagaagacaatgaaagtcacaggagtaactactcagggagtaaaatctctgcttaccagcatgtatgtgaaggagttcctcatctccagcagtcaagatggccatcagtggactctcttttttcagaatggcaaagtaaaggtttttcagggaaatcaagactccttcacacctgtggtgaactctctagacccaccgttactgactcgctaccttcgaattcacccccagagttgggtgcaccagattgccctgaggatggaggttctgggctgcgaggcacaggacctctac

SEQ ID NO: 20 - protein, 500 aa, Artificial
  linker
GGGGSGGGGSGGGGSGGGGSGGGGSGGGGSGGGGSGGGGSGGGGSGGGGSGGGGSGGGGSGGGGSGGGGSGGGGSGGGGSGGGGSGGGGSGGGGSGGGGSGGGGSGGGGSGGGGSGGGGSGGGGSGGGGSGGGGSGGGGSGGGGSGGGGSGGGGSGGGGSGGGGSGGGGSGGGGSGGGGSGGGGSGGGGSGGGGSGGGGSGGGGSGGGGSGGGGSGGGGSGGGGSGGGGSGGGGSGGGGSGGGGSGGGGSGGGGSGGGGSGGGGSGGGGSGGGGSGGGGSGGGGSGGGGSGGGGSGGGGSGGGGSGGGGSGGGGSGGGGSGGGGSGGGGSGGGGSGGGGSGGGGSGGGGSGGGGSGGGGSGGGGSGGGGSGGGGSGGGGSGGGGSGGGGSGGGGSGGGGSGGGGSGGGGSGGGGSGGGGSGGGGSGGGGSGGGGSGGGGSGGGGSGGGGSGGGGSGGGGSGGGGSGGGGSGGGGSGGGGSGGGGSGGGGSGGGGSGGGGS

SEQ ID NO: 21 - protein, 800 aa, Artificial
  linker
  REPEAT (1)..(300): Gly-Gly-Ser repeats 1 to 100 times
  REPEAT (301)..(800): Gly-Gly-Gly-Gly-Ser repeats 1 to 100 times
GGSGGSGGSGGSGGSGGSGGSGGSGGSGGSGGSGGSGGSGGSGGSGGSGGSGGSGGSGGSGGSGGSGGSGGSGGSGGSGGSGGSGGSGGSGGSGGSGGSGGSGGSGGSGGSGGSGGSGGSGGSGGSGGSGGSGGSGGSGGSGGSGGSGGSGGSGGSGGSGGSGGSGGSGGSGGSGGSGGSGGSGGSGGSGGSGGSGGSGGSGGSGGSGGSGGSGGSGGSGGSGGSGGSGGSGGSGGSGGSGGSGGSGGSGGSGGSGGSGGSGGSGGSGGSGGSGGSGGSGGSGGSGGSGGSGGSGGSGGSGGGGSGGGGSGGGGSGGGGSGGGGSGGGGSGGGGSGGGGSGGGGSGGGGSGGGGSGGGGSGGGGSGGGGSGGGGSGGGGSGGGGSGGGGSGGGGSGGGGSGGGGSGGGGSGGGGSGGGGSGGGGSGGGGSGGGGSGGGGSGGGGSGGGGSGGGGSGGGGSGGGGSGGGGSGGGGSGGGGSGGGGSGGGGSGGGGSGGGGSGGGGSGGGGSGGGGSGGGGSGGGGSGGGGSGGGGSGGGGSGGGGSGGGGSGGGGSGGGGSGGGGSGGGGSGGGGSGGGGSGGGGSGGGGSGGGGSGGGGSGGGGSGGGGSGGGGSGGGGSGGGGSGGGGSGGGGSGGGGSGGGGSGGGGSGGGGSGGGGSGGGGSGGGGSGGGGSGGGGSGGGGSGGGGSGGGGSGGGGSGGGGSGGGGSGGGGSGGGGSGGGGSGGGGSGGGGSGGGGSGGGGSGGGGSGGGGSGGGGSGGGGSGGGGSGGGGSGGGGSGGGGSGGGGSGGGGSGGGGS

SEQ ID NO: 22 - protein, 7 aa, Artificial
  linker
SGGSGGS

SEQ ID NO: 23 - protein, 15 aa, Artificial
  linker
GGSGGSGGSGGSGGG

SEQ ID NO: 24 - protein, 16 aa, Artificial
  linker
GGSGGSGGGGSGGGGS

SEQ ID NO: 25 - protein, 18 aa, Artificial
  linker
GGSGGSGGSGGSGGSGGS

SEQ ID NO: 26 - protein, 15 aa, Artificial
  linker
  REPEAT (1)..(15): Gly-Gly-Gly-Gly-Ser repeats 1 to 3 times
GGGGSGGGGSGGGGS

SEQ ID NO: 27 - protein, 100 aa, Artificial
  linker
  REPEAT (1)..(100): Gly-Gly-Gly-Gly-Ser repeats 1 to 20 times
GGGGSGGGGSGGGGSGGGGSGGGGSGGGGSGGGGSGGGGSGGGGSGGGGSGGGGSGGGGSGGGGSGGGGSGGGGSGGGGSGGGGSGGGGSGGGGSGGGGS

SEQ ID NO: 28 - protein, 15 aa, Artificial
  linker
  REPEAT (1)..(15): Gly-Gly-Gly-Gly-Ser is repeated 1 to 3 times
GGGGSGGGGSGGGGS

SEQ ID NO: 29 - protein, 7 aa, Artificial
  cleavable linker
  MISC_FEATURE (4)..(5): FXIa cleavage site
KLTRAET

SEQ ID NO: 30 - protein, 7 aa, Artificial
  cleavable linker
  MISC_FEATURE (4)..(5): FXIa cleavage site
DFTRVVG

SEQ ID NO: 31 - protein, 8 aa, Artificial
  cleavable linker
  MISC_FEATURE (4)..(5): FXIIa cleavage site
TMTRIVGG

SEQ ID NO: 32 - protein, 8 aa, Artificial
  cleavable linker
  MISC_FEATURE (4)..(5): Kallikrein cleavage site
SPFRSTGG

SEQ ID NO: 33 - protein, 8 aa, Artificial
  cleavable linker
  misc_feature (4)..(5): FVIIa cleavage site
LQVRIVGG

SEQ ID NO: 34 - protein, 8 aa, Artificial
  cleavable linker
  misc_feature (4)..(5): FIXa cleavage site
PLGRIVGG

SEQ ID NO: 35 - protein, 8 aa, Artificial
  cleavable linker
  misc_feature (4)..(5): FXa cleavage site
IEGRTVGG

SEQ ID NO: 36 - protein, 8 aa, Artificial
  cleavable linker
  misc_feature (4)..(5): FIIa (thrombin) cleavage site
LTPRSLLV

SEQ ID NO: 37 - protein, 8 aa, Artificial
  cleavable linker
  misc_feature (4)..(5): Elastase-2 cleavage site
LGPVSGVP

SEQ ID NO: 38 - protein, 8 aa, Artificial
  cleavable linker
  misc_feature (4)..(5): Granzyme-B cleavage site
VAGDSLEE

SEQ ID NO: 39 - protein, 8 aa, Artificial
  cleavable linker
  misc_feature (4)..(5): MMP-12 cleavage site
GPAGLGGA

SEQ ID NO: 40 - protein, 8 aa, Artificial
  cleavable linker
  misc_feature (4)..(5): MMP-13 cleavage site
GPAGLRGA

SEQ ID NO: 41 - protein, 8 aa, Artificial
  cleavable linker
  misc_feature (4)..(5): MMP-17 cleavage site
APLGLRLR

SEQ ID NO: 42 - protein, 8 aa, Artificial
  cleavable linker
  misc_feature (4)..(5): MMP-20 cleavage site
PALPLVAQ

SEQ ID NO: 43 - protein, 7 aa, Artificial
  cleavable linker
  misc_feature (6)..(7): TEV cleavage site
ENLYFQG

SEQ ID NO: 44 - protein, 8 aa, Artificial
  cleavable linker
  misc_feature (4)..(5): Enterokinase cleavage site
DDDKIVGG

SEQ ID NO: 45 - protein, 8 aa, Artificial
  cleavable linker
  misc_feature (6)..(7): Protease C (PRESCISSION) cleavage site
LEVLFQGP

SEQ ID NO: 46 - protein, 8 aa, Artificial
  cleavable linker
  misc_feature (4)..(5): Sortase A
LPKTGSES

SEQ ID NO: 47 - protein, 9 aa, Artificial
  cleavable linker
TQSFNDFTR

SEQ ID NO: 48 - protein, 10 aa, Artificial
  cleavage site
SVSQTSKLTR

SEQ ID NO: 49 - protein, 10 aa, Artificial
  cleavage site
DFLAEGGGVR

SEQ ID NO: 50 - protein, 7 aa, Artificial
  cleavage site
TTKIKPR

SEQ ID NO: 51 - protein, 10 aa, Artificial
  cleavge site
ALRPRVVGGA

SEQ ID NO: 52 - protein, 4 aa, Artificial
  cleavage site
RRRR

SEQ ID NO: 53 - protein, 6 aa, Artificial
  cleavage site
RKRRKR

SEQ ID NO: 54 - protein, 5 aa, Artificial
  cleavage site
RRRRS

SEQ ID NO: 55 - protein, 5 aa, Artificial
  cleavage site
LVPRG

SEQ ID NO: 56 - protein, 25 aa, Artificial
  cleavage and linker site
TLDPRSFLLRNPNDKYEPFWEDEEK

SEQ ID NO: 57 - DNA, 99 bp, Artificial
  ESC48-Fwd-VWF-D'D3 with VIII signal and BsiW1 site for pSYN VWF-001
tcgcgacgtacggccgccaccatgcaaatagagctctccacctgcttctttctgtgccttttgcgattctgctttagcctatcctgtcggccccccatg

SEQ ID NO: 58 - DNA, 68 bp, Artificial
  ESC50- Rev- VWF- partial D'D3 (1-276 amino acid) with 6 His and Not1 site for pSYN VWF- 001
tgacctcgagcggccgctcagtggtgatggtgatgatgcagaggcacttttctggtgtcagcacactg

SEQ ID NO: 59 - DNA, 99 bp, Artificial; identical to SEQ ID NO: 57
  ESC48- Fwd - VWF-D'D3 with VIII signal and BsiW1 site for pSYN VWF- 002

SEQ ID NO: 60 - DNA, 71 bp, Artificial
  ESC51- Rev- VWF D'D3 (1-477 amino acid) with 6His and Not 1 site for pSYN VWF- 002
tgacctcgagcggccgctcagtggtgatggtgatgatgcctgctgcagtagaaatcgtgcaacggcggttc

SEQ ID NO: 61 - DNA, 99 bp, Artificial; identical to SEQ ID NO: 57
  ESC48- Fwd - VWF-D'D3 with VIII signal and BsiW1 site for pSYN VWF- 003

SEQ ID NO: 62 - DNA, 65 bp, Artificial
  ESC52- Rev-VWF-D'D3 Partial A1 (1-511 amino acids) with 6His and Not1 site for pSYN VWF- 003
tgacctcgagcggccgctcagtggtgatggtgatgatggcccacagtgacttgtgccatgtgggg

SEQ ID NO: 63 - DNA, 99 bp, Artificial; identical to SEQ ID NO: 57
  ESC48- Fwd - VWF-D'D3 with VIII signal and BsiW1 site for pSYN VWF- 004

SEQ ID NO: 64 - DNA, 65 bp, Artificial; identical to SEQ ID NO: 62
  ESC53-Rev- VWF-D'D3A1 (1-716 amino acids) with 6His and Not1 site for pSYN VWF- 004

SEQ ID NO: 65 - DNA, 1313 bp, Artificial
  cloned vector
ggatcctagtggggaataagggatgcagccacccctcagtgaaatgcaagaaacgggtcaccatcctggtggagggaggagagattgagctgtttgacggggaggtgaatgtgaagaggcccatgaaggatgagactcactttgaggtggtggagtctggccggtacatcattctgctgctgggcaaagccctctccgtggtctgggaccgccacctgagcatctccgtggtcctgaagcagacataccaggagaaagtgtgtggcctgtgtgggaattttgatggcatccagaacaatgacctcaccagcagcaacctccaagtggaggaagaccctgtggactttgggaactcctggaaagtgagctcgcagtgtgctgacaccagaaaagtgcctctggactcatcccctgccacctgccataacaacatcatgaagcagacgatggtggattcctcctgtagaatccttaccagtgacgtcttccaggactgcaacaagctggtggaccccgagccatatctggatgtctgcatttacgacacctgctcctgtgagtccattggggactgcgcctgcttctgcgacaccattgctgcctatgcccacgtgtgtgcccagcatggcaaggtggtgacctggaggacggccacattgtgcccccagagctgcgaggagaggaatctccgggagaacgggtatgagtgtgagtggcgctataacagctgtgcacctgcctgtcaagtcacgtgtcagcaccctgagccactggcctgccctgtgcagtgtgtggagggctgccatgcccactgccctccagggaaaatcctggatgagcttttgcagacctgcgttgaccctgaagactgtccagtgtgtgaggtggctggccggcgttttgcctcaggaaagaaagtcaccttgaatcccagtgaccctgagcactgccagatttgccactgtgatgttgtcaacctcacctgtgaagcctgccaggagccgggaggcctggtggtgcctcccacagatgccccggtgagccccaccactctgtatgtggatgagacgctccaggatggctgtgatactcacttctgcaaggtcaatgagagaggagagtacttctgggagaagagggtcacaggctgcccaccctttgatgaacacaagtgtcttgctgagggaggtaaaattatgaaaattccaggcacctgctgtgacacatgtgaggagcctgagtgcaacgacatcactgccaggctgcagtatgtcaaggtgggaagctgtaagtctgaagtagaggtggatatc

SEQ ID NO: 66 - DNA, 32 bp, Artificial
  ESC 89-fwd with Nhe1site
ctcactatagggagacccaagctggctagccg

SEQ ID NO: 67 - DNA, 43 bp, Artificial
  ESC 91-rev with Sal1
ctggatcccgggagtcgactcgtcagtggtgatggtgatgatg

SEQ ID NO: 68 - DNA, 92 bp, Artificial
  LW 22-FWD-VWF-D'D3 with FVIII signal sequence and BsiW1 site
gcgccggccgtacgatgcaaatagagctctccacctgcttctttctgtgccttttgcgattctgctttagcctatcctgtcggccccccatg

SEQ ID NO: 69 - DNA, 47 bp, Artificial
  LW 23-Rev- Fc with stop codon and Not1 site
tcatcaatgtatcttatcatgtctgaattcgcggccgctcatttacc

SEQ ID NO: 70 - DNA, 41 bp, Artificial
  LW24- Fwd- VWF D1D2D'D3 cloning oligo with BsiW1 site
gcgccggccgtacgatgattcctgccagatttgccggggtg

SEQ ID NO: 71 - DNA, 41 bp, Artificial
  LW27-Rev-VWF  D'D3 oligo with EcoRV
ccaccgccagatatcggctcctggcaggcttcacaggtgag

SEQ ID NO: 72 - protein, 1240 aa, Artificial
  VWF-D1D2D'D3
MIPARFAGVLLALALILPGTLCAEGTRGRSSTARCSLFGSDFVNTFDGSMYSFAGYCSYLLAGGCQKRSFSIIGDFQNGKRVSLSVYLGEFFDIHLFVNGTVTQGDQRVSMPYASKGLYLETEAGYYKLSGEAYGFVARIDGSGNFQVLLSDRYFNKTCGLCGNFNIFAEDDFMTQEGTLTSDPYDFANSWALSSGEQWCERASPPSSSCNISSGEMQKGLWEQCQLLKSTSVFARCHPLVDPEPFVALCEKTLCECAGGLECACPALLEYARTCAQEGMVLYGWTDHSACSPVCPAGMEYRQCVSPCARTCQSLHINEMCQERCVDGCSCPEGQLLDEGLCVESTECPCVHSGKRYPPGTSLSRDCNTCICRNSQWICSNEECPGECLVTGQSHFKSFDNRYFTFSGICQYLLARDCQDHSFSIVIETVQCADDRDAVCTRSVTVRLPGLHNSLVKLKHGAGVAMDGQDIQLPLLKGDLRIQHTVTASVRLSYGEDLQMDWDGRGRLLVKLSPVYAGKTCGLCGNYNGNQGDDFLTPSGLAEPRVEDFGNAWKLHGDCQDLQKQHSDPCALNPRMTRFSEEACAVLTSPTFEACHRAVSPLPYLRNCRYDVCSCSDGRECLCGALASYAAACAGRGVRVAWREPGRCELNCPKGQVYLQCGTPCNLTCRSLSYPDEECNEACLEGCFCPPGLYMDERGDCVPKAQCPCYYDGEIFQPEDIFSDHHTMCYCEDGFMHCTMSGVPGSLLPDAVLSSPLSHRSKRSLSCRPPMVKLVCPADNLRAEGLECTKTCQNYDLECMSMGCVSGCLCPPGMVRHENRCVALERCPCFHQGKEYAPGETVKIGCNTCVCRDRKWNCTDHVCDATCSTIGMAHYLTFDGLKYLFPGECQYVLVQDYCGSNPGTFRILVGNKGCSHPSVKCKKRVTILVEGGEIELFDGEVNVKRPMKDETHFEVVESGRYIILLLGKALSVVWDRHLSISVVLKQTYQEKVCGLCGNFDGIQNNDLTSSNLQVEEDPVDFGNSWKVSSQCADTRKVPLDSSPATCHNNIMKQTMVDSSCRILTSDVFQDCNKLVDPEPYLDVCIYDTCSCESIGDCACFCDTIAAYAHVCAQHGKVVTWRTATLCPQSCEERNLRENGYECEWRYNSCAPACQVTCQHPEPLACPVQCVEGCHAHCPPGKILDELLQTCVDPEDCPVCEVAGRRFASGKKVTLNPSDPEHCQICHCDVVNLTCEACQEP

SEQ ID NO: 73 - protein, 477 aa, Artificial
  VWF-D'D3
SLSCRPPMVKLVCPADNLRAEGLECTKTCQNYDLECMSMGCVSGCLCPPGMVRHENRCVALERCPCFHQGKEYAPGETVKIGCNTCVCRDRKWNCTDHVCDATCSTIGMAHYLTFDGLKYLFPGECQYVLVQDYCGSNPGTFRILVGNKGCSHPSVKCKKRVTILVEGGEIELFDGEVNVKRPMKDETHFEVVESGRYIILLLGKALSVVWDRHLSISVVLKQTYQEKVCGLCGNFDGIQNNDLTSSNLQVEEDPVDFGNSWKVSSQCADTRKVPLDSSPATCHNNIMKQTMVDSSCRILTSDVFQDCNKLVDPEPYLDVCIYDTCSCESIGDCACFCDTIAAYAHVCAQHGKVVTWRTATLCPQSCEERNLRENGYECEWRYNSCAPACQVTCQHPEPLACPVQCVEGCHAHCPPGKILDELLQTCVDPEDCPVCEVAGRRFASGKKVTLNPSDPEHCQICHCDVVNLTCEACQEP

SEQ ID NO: 74 - protein, 30 aa, Artificial
  VWF-D'D3 domain (1-477aa; C336A/C379A mutation)
  REPEAT (1)..(30): Gly-Gly-Gly-Gly-Ser repeats 6 times
GGGGSGGGGSGGGGSGGGGSGGGGSGGGGS

SEQ ID NO: 75 - protein, 5 aa, Artificial
  linker
RRRRS

SEQ ID NO: 76 - protein, 6 aa, Artificial
  linker
RKRRKR

SEQ ID NO: 77 - DNA, 24 bp, Artificial
  ESC17-Fwd- VWF cloning oligo with Cla1
gtccggcatgagaatcgatgtgtg

SEQ ID NO: 78 - DNA, 31 bp, Artificial
  ESC41- Rev-VWF with EcoRV
cctccaccgccagatatcagaggcacttttc

SEQ ID NO: 79 - DNA, 105 bp, Artificial
  ESC78- Fwd with EcoRV site
aaagtgcctctgatatctggcggtggaggttccggtggcgggggatccggtggcgggggatccggtggcgggggatccggtggcgggggatccctggtcccccgg

SEQ ID NO: 80 - DNA, 107 bp, Artificial
  ESC79- Rev with RsRII site
gaagaggaagactgacggtccgcccaggagttctggagctgggcacggtgggcatgtgtgagttttgtcgcctccgctgccccgggggaccagggatcccccgccac

SEQ ID NO: 81 - protein, 48 aa, Artificial
  linker
ISGGGGSGGGGSGGGGSGGGGSGGGGSGGGGSLVPRGSGGGGSGGGGS

SEQ ID NO: 82 - DNA, 1781 bp, Artificial
  pSYN-FVIII-049, which is FVIII-Fc construct with a cleavable linker in between two Fc domains; Genscript-Sequence number 103069
ccgtcgacaagagcaggtggcagcaggggaacgtcttctcatgctccgtgatgcatgaggctctgcacaaccactacacgcagaagagcctctccctgtctccgggtaaacggcgccgccggagcggtggcggcggatcaggtgggggtggatcaggcggtggaggttccggtggcgggggatccggcggtggaggttccggtgggggtggatcaaggaagaggaggaagagaagcctatcctgtcggccccccatggtcaagctggtgtgtcccgctgacaacctgcgggctgaagggctcgagtgtaccaaaacgtgccagaactatgacctggagtgcatgagcatgggctgtgtctctggctgcctctgccccccgggcatggtccggcatgagaatcgatgtgtggccctggaaaggtgtccctgcttccatcagggcaaggagtatgcccctggagaaacagtgaagattggctgcaacacttgtgtctgtcgggaccggaagtggaactgcacagaccatgtgtgtgatgccacgtgctccacgatcggcatggcccactacctcaccttcgacgggctcaaatacctgttccccggggagtgccagtacgttctggtgcaggattactgcggcagtaaccctgggacctttcggatcctagtggggaataagggatgcagccacccctcagtgaaatgcaagaaacgggtcaccatcctggtggagggaggagagattgagctgtttgacggggaggtgaatgtgaagaggcccatgaaggatgagactcactttgaggtggtggagtctggccggtacatcattctgctgctgggcaaagccctctccgtggtctgggaccgccacctgagcatctccgtggtcctgaagcagacataccaggagaaagtgtgtggcctgtgtgggaattttgatggcatccagaacaatgacctcaccagcagcaacctccaagtggaggaagaccctgtggactttgggaactcctggaaagtgagctcgcagtgtgctgacaccagaaaagtgcctctggactcatcccctgccacctgccataacaacatcatgaagcagacgatggtggattcctcctgtagaatccttaccagtgacgtcttccaggactgcaacaagctggtggaccccgagccatatctggatgtctgcatttacgacacctgctcctgtgagtccattggggactgcgccgcattctgcgacaccattgctgcctatgcccacgtgtgtgcccagcatggcaaggtggtgacctggaggacggccacattgtgcccccagagctgcgaggagaggaatctccgggagaacgggtatgaggctgagtggcgctataacagctgtgcacctgcctgtcaagtcacgtgtcagcaccctgagccactggcctgccctgtgcagtgtgtggagggctgccatgcccactgccctccagggaaaatcctggatgagcttttgcagacctgcgttgaccctgaagactgtccagtgtgtgaggtggctggccggcgttttgcctcaggaaagaaagtcaccttgaatcccagtgaccctgagcactgccagatttgccactgtgatgttgtcaacctcacctgtgaagcctgccaggagccgatcgatggcggtggaggttccggtggcgggggatccctggtcccccggggcagcggaggcgacaaaactcacacatgcccaccgtgcccagctccagaactcctgggcggaccgtca

SEQ ID NO: 83 - DNA, 220 bp, Artificial
  A fragment of the Genscript construct was sub cloned into the EcoRV/RsRII digested pSYN-FVIII-0159; Genscript-Sequence no-132601
aaagtgcctctgatatctggcggtggaggttccggtggcgggggatccggcggtggaggttccggcggtggaggttccggtggcgggggatccggtggcgggggatccctggtcccccggggcagcggcggtggaggttccggtggcgggggatccgacaaaactcacacatgcccaccgtgcccagctccagaactcctgggcggaccgtcagtcttcc

SEQ ID NO: 84 - protein, 73 aa, Artificial
  pSYN-VIII-178 has a 73 amino acids linker in between the VWF fragment and the Fc region; synthesis of DNA fragment coding for 73 amino acids linker
ISGGGGSGGGGSGGGGSGGGGSGGGGSGGGGSGGGGSGGGGSGGGGSGGGGSGGGGSLVPRGSGGGGSGGGGS

SEQ ID NO: 85 - DNA, 299 bp, Artificial
  Genscript-Sequence #-144849
gcctgccaggagccgatatctggcggtggaggttccggtggcgggggatccggcggtggaggttccggcggtggaggttccggtggcgggggatccggcggtggaggttccggtggcgggggatccggcggtggaggttccggcggtggaggttccggtggcgggggatccggtggcgggggatccctggtcccccggggcagcggcggtggaggttccggtggcgggggatccgacaaaactcacacatgcccccgtgcccagctccagaactcctgggcggaccgtcagtcttcctc

SEQ ID NO: 86 - protein, 98 aa, Artificial
  linker
ISGGGGSGGGGSGGGGSGGGGSGGGGSGGGGSGGGGSGGGGSGGGGSGGGGSGGGGSGGGGSGGGGSGGGGSGGGGSGGGGSLVPRGSGGGGSGGGGS

SEQ ID NO: 87 - DNA, 380 bp, Artificial
  Genscript-Sequence #-144849
gcctgccaggagccgatatctggcggtggaggttccggtggcgggggatccggcggtggaggttccggcggtggaggttccggtggcgggggatccggcggtggaggttccggtggcgggggatccggcggtggaggttccggcggtggaggttccggtggcgggggatccggcggtggaggttccggtggcgggggatccggcggtggaggttccggcggtggaggttccggtggcgggggatccggtggcgggggatccctggtcccccggggcagcggcggtggaggttccggtggcgggggatccgacaaaactcacacatgcccaccgtgcccagctccagaactcctgggcggaccgtcagtcttcctcttccc

SEQ ID NO: 88 - protein, 2449 aa, Artificial [sequence omitted]

SEQ ID NO: 89 - protein, 48 aa, Artificial; identical to SEQ ID NO: 81
  a 48-amino acid linker

SEQ ID NO: 90 - protein, 1665 aa, Artificial
  pSYN-FVIII-155 mature protein
ATRRYYLGAVELSWDYMQSDLGELPVDARFPPRVPKSFPFNTSVVYKKTLFVEFTDHLFNIAKPRPPWMGLLGPTIQAEVYDTVVITLKNMASHPVSLHAVGVSYWKASEGAEYDDQTSQREKEDDKVFPGGSHTYVWQVLKENGPMASDPLCLTYSYLSHVDLVKDLNSGLIGALLVCREGSLAKEKTQTLHKFILLFAVFDEGKSWHSETKNSLMQDRDAASARAWPKMHTVNGYVNRSLPGLIGCHRKSVYWHVIGMGTTPEVHSIFLEGHTFLVRNHRQASLEISPITFLTAQTLLMDLGQFLLFCHISSHQHDGMEAYVKVDSCPEEPQLRMKNNEEAEDYDDDLTDSEMDVVRFDDDNSPSFIQIRSVAKKHPKTWVHYIAAEEEDWDYAPLVLAPDDRSYKSQYLNNGPQRIGRKYKKVRFMAYTDETFKTREAIQHESGILGPLLYGEVGDTLLIIFKNQASRPYNIYPHGITDVRPLYSRRLPKGVKHLKDFPILPGEIFKYKWTVTVEDGPTKSDPRCLTRYYSSFVNMERDLASGLIGPLLICYKESVDQRGNQIMSDKRNVILFSVFDENRSWYLTENIQRFLPNPAGVQLEDPEFQASNIMHSINGYVFDSLQLSVCLHEVAYWYILSIGAQTDFLSVFFSGYTFKHKMVYEDTLTLFPFSGETVFMSMENPGLWILGCHNSDFRNRGMTALLKVSSCDKNTGDYYEDSYEDISAYLLSKNNAIEPRSFSQNPPVLKAHQAEITRTTLQSDQEEIDYDDTISVEMKKEDFDIYDEDENQSPRSFQKKTRHYFIAAVERLWDYGMSSSPHVLRNRAQSGSVPQFKKVVFQEFTDGSFTQPLYRGELNEHLGLLGPYIRAEVEDNIMVTFRNQASRPYSFYSSLISYEEDQRQGAEPRKNFVKPNETKTYFWKVQHHMAPTKDEFDCKAWAYFSDVDLEKDVHSGLIGPLLVCHTNTLNPAHGRQVTVQEFALFFTIFDETKSWYFTENMERNCRAPCNIQMEDPTFKENYRFHAINGYIMDTLPGLVMAQDQRIRWYLLSMGSNENIHSIHFSGHVFTVRKKEEYKMALYNLYPGVFETVEMLPSKAGIWRVECLIGEHLHAGMSTLFLVYSNKCQTPLGMASGHIRDFQITASGQYGQWAPKLARLHYSGSINAWSTKEPFSWIKVDLLAPMIIHGIKTQGARQKFSSLYISQFIIMYSLDGKKWQTYRGNSTGTLMVFFGNVDSSGIKHNIFNPPIIARYIRLHPTHYSIRSTLRMELMGCDLNSCSMPLGMESKAISDAQITASSYFTNMFATWSPSKARLHLQGRSNAWRPQVNNPKEWLQVDFQKTMKVTGVTTQGVKSLLTSMYVKEFLISSSQDGHQWTLFFQNGKVKVFQGNQDSFTPVVNSLDPPLLTRYLRIHPQSWVHQIALRMEVLGCEAQDLYDKTHTCPPCPAPELLGGPSVFLFPPKPKDTLMISRTPEVTCVVVDVSHEDPEVKFNWYVDGVEVHNAKTKPREEQYNSTYRVVSVLTVLHQDWLNGKEYKCKVSNKALPAPIEKTISKAKGQPREPQVYTLPPSRDELTKNQVSLTCLVKGFYPSDIAVEWESNGQPENNYKTTPPVLDSDGSFFLYSKLTVDKSRWQQGNVFSCSVMHEALHNHYTQKSLSLSPGK

SEQ ID NO: 91 - DNA, 5052 bp, Artificial
  pSYN-FVIII-155
atgcaaatagagctctccacctgcttctttctgtgccttttgcgattctgctttagtgccaccagaagatactacctgggtgcagtggaactgtcatgggactatatgcaaagtgatctcggtgagctgcctgtggacgcaagatttcctcctagagtgccaaaatcttttccattcaacacctcagtcgtgtacaaaaagactctgtttgtagaattcacggatcaccttttcaacatcgctaagccaaggccaccctggatgggtctgctaggtcctaccatccaggctgaggtttatgatacagtggtcattacacttaagaacatggcttcccatcctgtcagtcttcatgctgttggtgtatcctactggaaagcttctgagggagctgaatatgatgatcagaccagtcaaagggagaaagaagatgataaagtcttccctggtggaagccatacatatgtctggcaggtcctgaaagagaatggtccaatggcctctgacccactgtgccttacctactcatatctttctcatgtggacctggtaaaagacttgaattcaggcctcattggagccctactagtatgtagagaagggagtctggccaaggaaaagacacagaccttgcacaaatttatactactttttgctgtatttgatgaagggaaaagttggcactcagaaacaaagaactccttgatgcaggatagggatgctgcatctgctcgggcctggcctaaaatgcacacagtcaatggttatgtaaacaggtctctgccaggtctgattggatgccacaggaaatcagtctattggcatgtgattggaatgggcaccactcctgaagtgcactcaatattcctcgaaggtcacacatttcttgtgaggaaccatcgccaggcgtccttggaaatctcgccaataactttccttactgctcaaacactcttgatggaccttggacagtttctactgttttgtcatatctcttcccaccaacatgatggcatggaagcttatgtcaaagtagacagctgtccagaggaaccccaactacgaatgaaaaataatgaagaagcggaagactatgatgatgatcttactgattctgaaatggatgtggtcaggtttgatgatgacaactctccttcctttatccaaattcgctcagttgccaagaagcatcctaaaacttgggtacattacattgctgctgaagaggaggactgggactatgctcccttagtcctcgcccccgatgacagaagttataaaagtcaatatttgaacaatggccctcagcggattggtaggaagtacaaaaaagtccgatttatggcatacacagatgaaacctttaagactcgtgaagctattcagcatgaatcaggaatcttgggacctttactttatggggaagttggagacacactgttgattatatttaagaatcaagcaagcagaccatataacatctaccctcacggaatcactgatgtccgtcctttgtattcaaggagattaccaaaaggtgtaaaacatttgaaggattttccaattctgccaggagaaatattcaaatataaatggacagtgactgtagaagatgggccaactaaatcagatcctcggtgcctgacccgctattactctagtttcgttaatatggagagagatctagcttcaggactcattggccctctcctcatctgctacaaagaatctgtagatcaaagaggaaaccagataatgtcagacaagaggaatgtcatcctgttttctgtatttgatgagaaccgaagctggtacctcacagagaatatacaacgctttctccccaatccagctggagtgcagcttgaggatccagagttccaagcctccaacatcatgcacagcatcaatggctatgtttttgatagtttgcagttgtcagtttgtttgcatgaggtggcatactggtacattctaagcattggagcacagactgacttcctttctgtcttcttctctggatataccttcaaacacaaaatggtctatgaagacacactcaccctattcccattctcaggagaaactgtcttcatgtcgatggaaaacccaggtctatggattctggggtgccacaactcagactttcggaacagaggcatgaccgccttactgaaggtttctagttgtgacaagaacactggtgattattacgaggacagttatgaagatatttcagcatacttgctgagtaaaaacaatgccattgaaccaagaagcttctctcaaaacccaccagtcttgaaagcccatcaggcggaaataactcgtactactcttcagtcagatcaagaggaaattgactatgatgataccatatcagttgaaatgaagaaggaagattttgacatttatgatgaggatgaaaatcagagcccccgcagctttcaaaagaaaacacgacactattttattgctgcagtggagaggctctgggattatgggatgagtagctccccacatgttctaagaaacagggctcagagtggcagtgtccctcagttcaagaaagttgttttccaggaatttactgatggctcctttactcagcccttataccgtggagaactaaatgaacatttgggactcctggggccatatataagagcagaagttgaagataatatcatggtaactttcagaaatcaggcctctcgtccctattccttctattctagccttatttcttatgaggaagatcagaggcaaggagcagaacctagaaaaaactttgtcaagcctaatgaaaccaaaacttacttttggaaagtgcaacatcatatggcacccactaaagatgagtttgactgcaaagcctgggcttatttctctgatgttgacctggaaaaagatgtgcactcaggcctgattggaccccttctggtctgccacactaacacactgaaccctgctcatgggagacaagtgacagtacaggaatttgctctgtttttcaccatctttgatgagaccaaaagctggtacttcactgaaaatatggaaagaaactgcagggctccctgcaatatccagatggaagatcccacttttaaagagaattatcgcttccatgcaatcaatggctacataatggatacactacctggcttagtaatggctcaggatcaaaggattcgatggtatctgctcagcatgggcagcaatgaaaacatccattctattcatttcagtggacatgtgttcactgtacgaaaaaaagaggagtataaaatggcactgtacaatctctatccaggtgtttttgagacagtggaaatgttaccatccaaagctggaatttggcgggtggaatgccttattggcgagcatctacatgctgggatgagcacactttttctggtgtacagcaataagtgtcagactcccctgggaatggcttctggacacattagagattttcagattacagcttcaggacaatatggacagtgggccccaaagctggccagacttcattattccggatcaatcaatgcctggagcaccaaggagcccttttcttggatcaaggtggatctgttggcaccaatgattattcacggcatcaagacccagggtgcccgtcagaagttctccagcctctacatctctcagtttatcatcatgtatagtcttgatgggaagaagtggcagacttatcgaggaaattccactggaaccttaatggtcttctttggcaatgtggattcatctgggataaaacacaatatttttaaccctccaattattgctcgatacatccgtttgcacccaactcattatagcattcgcagcactcttcgcatggagttgatgggctgtgatttaaatagttgcagcatgccattgggaatggagagtaaagcaatatcagatgcacagattactgcttcatcctactttaccaatatgtttgccacctggtctccttcaaaagctcgacttcacctccaagggaggagtaatgcctggagacctcaggtgaataatccaaaagagtggctgcaagtggacttccagaagacaatgaaagtcacaggagtaactactcagggagtaaaatctctgcttaccagcatgtatgtgaaggagttcctcatctccagcagtcaagatggccatcagtggactctcttttttcagaatggcaaagtaaaggtttttcagggaaatcaagactccttcacacctgtggtgaactctctagacccaccgttactgactcgctaccttcgaattcacccccagagttgggtgcaccagattgccctgaggatggaggttctgggctgcgaggcacaggacctctacgacaaaactcacacatgcccaccgtgcccagctccagaactcctgggcggaccgtcagtcttcctcttccccccaaaacccaaggacaccctcatgatctcccggacccctgaggtcacatgcgtggtggtggacgtgagccacgaagaccctgaggtcaagttcaactggtacgtggacggcgtggaggtgcataatgccaagacaaagccgcgggaggagcagtacaacagcacgtaccgtgtggtcagcgtcctcaccgtcctgcaccaggactggctgaatggcaaggagtacaagtgcaaggtctccaacaaagccctcccagcccccatcgagaaaaccatctccaaagccaaagggcagccccgagaaccacaggtgtacaccctgcccccatcccgggatgagctgaccaagaaccaggtcagcctgacctgcctggtcaaaggcttctatcccagcgacatcgccgtggagtgggagagcaatgggcagccggagaacaactacaagaccacgcctcccgtgttggactccgacggctccttcttcctctacagcaagctcaccgtggacaagagcaggtggcagcaggggaacgtcttctcatgctccgtgatgcatgaggctctgcacaaccactacacgcagaagagcctctccctgtctccgggtaaa

SEQ ID NO: 92 - protein, 19 aa, Artificial
  GFVIII-159
IDGGGGSGGGGSLVPRGSG

SEQ ID NO: 93 - protein, 34 aa, Artificial
  GFVIII-160
ISGGGGSGGGGSGGGGSGGGGSGGGGSLVPRGSG

SEQ ID NO: 94 - protein, 48 aa, Artificial; identical to SEQ ID NO: 81
  FVIII-064

SEQ ID NO: 95 - protein, 48 aa, Artificial Sequence; identical to SEQ ID NO: 81
  VWF031

SEQ ID NO: 96 - protein, 73 aa, Artificial Sequence; identical to SEQ ID NO: 84
  VWF035

SEQ ID NO: 97 - protein, 98 aa, Artificial Sequence; identical to SEQ ID NO: 86
  VWF036

SEQ ID NO: 98 - protein, 54 aa, Artificial Sequence
  pSYN-VWF-051 linker
ISGGGGSGGGGSGGGGSGGGGSGGGGSGGGGSLPETGALRPRVVGGGGSGGGGS

SEQ ID NO: 99 - DNA, 232 bp, Artificial Sequence
  Genewiz-Sequence no-10-210746313
aggagccgatatctggcggtggaggttccggtggcgggggatccggcggtggaggttccggcggtggaggttccggtggcgggggatccggtggcgggggatccttacctgaaactggagccctgcggccccgggtcgtcggcggtggaggttccggtggcgggggatccgacaaaactcacacatgcccaccgtgcccagctccagaactcctgggcggaccgtcagtctt

SEQ ID NO: 100 - DNA, 4566 bp, Artificial Sequence
  pSYN-VWF051
atgattcctgccagatttgccggggtgctgcttgctctggccctcattttgccagggaccctttgtgcagaaggaactcgcggcaggtcatccacggcccgatgcagccttttcggaagtgacttcgtcaacacctttgatgggagcatgtacagctttgcgggatactgcagttacctcctggcagggggctgccagaaacgctccttctcgattattggggacttccagaatggcaagagagtgagcctctccgtgtatcttggggaattttttgacatccatttgtttgtcaatggtaccgtgacacagggggaccaaagagtctccatgccctatgcctccaaagggctgtatctagaaactgaggctgggtactacaagctgtccggtgaggcctatggctttgtggccaggatcgatggcagcggcaactttcaagtcctgctgtcagacagatacttcaacaagacctgcgggctgtgtggcaactttaacatctttgctgaagatgactttatgacccaagaagggaccttgacctcggacccttatgactttgccaactcatgggctctgagcagtggagaacagtggtgtgaacgggcatctcctcccagcagctcatgcaacatctcctctggggaaatgcagaagggcctgtgggagcagtgccagcttctgaagagcacctcggtgtttgcccgctgccaccctctggtggaccccgagccttttgtggccctgtgtgagaagactttgtgtgagtgtgctggggggctggagtgcgcctgccctgccctcctggagtacgcccggacctgtgcccaggagggaatggtgctgtacggctggaccgaccacagcgcgtgcagcccagtgtgccctgctggtatggagtataggcagtgtgtgtccccttgcgccaggacctgccagagcctgcacatcaatgaaatgtgtcaggagcgatgcgtggatggctgcagctgccctgagggacagctcctggatgaaggcctctgcgtggagagcaccgagtgtccctgcgtgcattccggaaagcgctaccctcccggcacctccctctctcgagactgcaacacctgcatttgccgaaacagccagtggatctgcagcaatgaagaatgtccaggggagtgccttgtcactggtcaatcccacttcaagagctttgacaacagatacttcaccttcagtgggatctgccagtacctgctggcccgggattgccaggaccactccttctccattgtcattgagactgtccagtgtgctgatgaccgcgacgctgtgtgcacccgctccgtcaccgtccggctgcctggcctgcacaacagccttgtgaaactgaagcatggggcaggagttgccatggatggccaggacatccagctccccctcctgaaaggtgacctccgcatccagcatacagtgacggcctccgtgcgcctcagctacggggaggacctgcagatggactgggatggccgcgggaggctgctggtgaagctgtcccccgtctatgccgggaagacctgcggcctgtgtgggaattacaatggcaaccagggcgacgacttccttaccccctctgggctggcggagccccgggtggaggacttcgggaacgcctggaagctgcacggggactgccaggacctgcagaagcagcacagcgatccctgcgccctcaacccgcgcatgaccaggttctccgaggaggcgtgcgcggtcctgacgtcccccacattcgaggcctgccatcgtgccgtcagcccgctgccctacctgcggaactgccgctacgacgtgtgctcctgctcggacggccgcgagtgcctgtgcggcgccctggccagctatgccgcggcctgcgcggggagaggcgtgcgcgtcgcgtggcgcgagccaggccgctgtgagctgaactgcccgaaaggccaggtgtacctgcagtgcgggaccccctgcaacctgacctgccgctctctctcttacccggatgaggaatgcaatgaggcctgcctggagggctgcttctgccccccagggctctacatggatgagaggggggactgcgtgcccaaggcccagtgcccctgttactatgacggtgagatcttccagccagaagacatcttctcagaccatcacaccatgtgctactgtgaggatggcttcatgcactgtaccatgagtggagtccccggaagcttgctgcctgacgctgtcctcagcagtcccctgtctcatcgcagcaaaaggagcctatcctgtcggccccccatggtcaagctggtgtgtcccgctgacaacctgcgggctgaagggctcgagtgtaccaaaacgtgccagaactatgacctggagtgcatgagcatgggctgtgtctctggctgcctctgccccccgggcatggtccggcatgagaacagatgtgtggccctggaaaggtgtccctgcttccatcagggcaaggagtatgcccctggagaaacagtgaagattggctgcaacacttgtgtctgtcgggaccggaagtggaactgcacagaccatgtgtgtgatgccacgtgctccacgatcggcatggcccactacctcaccttcgacgggctcaaatacctgttccccggggagtgccagtacgttctggtgcaggattactgcggcagtaaccctgggacctttcggatcctagtggggaataagggatgcagccacccctcagtgaaatgcaagaaacgggtcaccatcctggtggagggaggagagattgagctgtttgacggggaggtgaatgtgaagaggcccatgaaggatgagactcactttgaggtggtggagtctggccggtacatcattctgctgctgggcaaagccctctccgtggtctgggaccgccacctgagcatctccgtggtcctgaagcagacataccaggagaaagtgtgtggcctgtgtgggaattttgatggcatccagaacaatgacctcaccagcagcaacctccaagtggaggaagaccctgtggactttgggaactcctggaaagtgagctcgcagtgtgctgacaccagaaaagtgcctctggactcatcccctgccacctgccataacaacatcatgaagcagacgatggtggattcctcctgtagaatccttaccagtgacgtcttccaggactgcaacaagctggtggaccccgagccatatctggatgtctgcatttacgacacctgctcctgtgagtccattggggactgcgccgcattctgcgacaccattgctgcctatgcccacgtgtgtgcccagcatggcaaggtggtgacctggaggacggccacattgtgcccccagagctgcgaggagaggaatctccgggagaacgggtatgaggctgagtggcgctataacagctgtgcacctgcctgtcaagtcacgtgtcagcaccctgagccactggcctgccctgtgcagtgtgtggagggctgccatgcccactgccctccagggaaaatcctggatgagcttttgcagacctgcgttgaccctgaagactgtccagtgtgtgaggtggctggccggcgttttgcctcaggaaagaaagtcaccttgaatcccagtgaccctgagcactgccagatttgccactgtgatgttgtcaacctcacctgtgaagcctgccaggagccgatatctggcggtggaggttccggtggcgggggatccggcggtggaggttccggcggtggaggttccggtggcgggggatccggtggcgggggatccttacctgaaactggagccctgcggccccgggtcgtcggcggtggaggttccggtggcgggggatccgacaaaactcacacatgcccaccgtgcccagctccagaactcctgggcggaccgtcagtcttcctcttccccccaaaacccaaggacaccctcatgatctcccggacccctgaggtcacatgcgtggtggtggacgtgagccacgaagaccctgaggtcaagttcaactggtacgtggacggcgtggaggtgcataatgccaagacaaagccgcgggaggagcagtacaacagcacgtaccgtgtggtcagcgtcctcaccgtcctgcaccaggactggctgaatggcaaggagtacaagtgcaaggtctccaacaaagccctcccagcccccatcgagaaaaccatctccaaagccaaagggcagccccgagaaccacaggtgtacaccctgcccccatcccgggatgagctgaccaagaaccaggtcagcctgacctgcctggtcaaaggcttctatcccagcgacatcgccgtggagtgggagagcaatgggcagccggagaacaactacaagaccacgcctcccgtgttggactccgacggctccttcttcctctacagcaagctcaccgtggacaagagcaggtggcagcaggggaacgtcttctcatgctccgtgatgcatgaggctctgcacaaccactacacgcagaagagcctctccctgtctccgggtaaatga

SEQ ID NO: 101 - protein, 1521 aa, Artificial Sequence
  VWF051
MIPARFAGVLLALALILPGTLCAEGTRGRSSTARCSLFGSDFVNTFDGSMYSFAGYCSYLLAGGCQKRSFSIIGDFQNGKRVSLSVYLGEFFDIHLFVNGTVTQGDQRVSMPYASKGLYLETEAGYYKLSGEAYGFVARIDGSGNFQVLLSDRYFNKTCGLCGNFNIFAEDDFMTQEGTLTSDPYDFANSWALSSGEQWCERASPPSSSCNISSGEMQKGLWEQCQLLKSTSVFARCHPLVDPEPFVALCEKTLCECAGGLECACPALLEYARTCAQEGMVLYGWTDHSACSPVCPAGMEYRQCVSPCARTCQSLHINEMCQERCVDGCSCPEGQLLDEGLCVESTECPCVHSGKRYPPGTSLSRDCNTCICRNSQWICSNEECPGECLVTGQSHFKSFDNRYFTFSGICQYLLARDCQDHSFSIVIETVQCADDRDAVCTRSVTVRLPGLHNSLVKLKHGAGVAMDGQDIQLPLLKGDLRIQHTVTASVRLSYGEDLQMDWDGRGRLLVKLSPVYAGKTCGLCGNYNGNQGDDFLTPSGLAEPRVEDFGNAWKLHGDCQDLQKQHSDPCALNPRMTRFSEEACAVLTSPTFEACHRAVSPLPYLRNCRYDVCSCSDGRECLCGALASYAAACAGRGVRVAWREPGRCELNCPKGQVYLQCGTPCNLTCRSLSYPDEECNEACLEGCFCPPGLYMDERGDCVPKAQCPCYYDGEIFQPEDIFSDHHTMCYCEDGFMHCTMSGVPGSLLPDAVLSSPLSHRSKRSLSCRPPMVKLVCPADNLRAEGLECTKTCQNYDLECMSMGCVSGCLCPPGMVRHENRCVALERCPCFHQGKEYAPGETVKIGCNTCVCRDRKWNCTDHVCDATCSTIGMAHYLTFDGLKYLFPGECQYVLVQDYCGSNPGTFRILVGNKGCSHPSVKCKKRVTILVEGGEIELFDGEVNVKRPMKDETHFEVVESGRYIILLLGKALSVVWDRHLSISVVLKQTYQEKVCGLCGNFDGIQNNDLTSSNLQVEEDPVDFGNSWKVSSQCADTRKVPLDSSPATCHNNIMKQTMVDSSCRILTSDVFQDCNKLVDPEPYLDVCIYDTCSCESIGDCAAFCDTIAAYAHVCAQHGKVVTWRTATLCPQSCEERNLRENGYEAEWRYNSCAPACQVTCQHPEPLACPVQCVEGCHAHCPPGKILDELLQTCVDPEDCPVCEVAGRRFASGKKVTLNPSDPEHCQICHCDVVNLTCEACQEPISGGGGSGGGGSGGGGSGGGGSGGGGSGGGGSLPETGALRPRVVGGGGSGGGGSDKTHTCPPCPAPELLGGPSVFLFPPKPKDTLMISRTPEVTCVVVDVSHEDPEVKFNWYVDGVEVHNAKTKPREEQYNSTYRVVSVLTVLHQDWLNGKEYKCKVSNKALPAPIEKTISKAKGQPREPQVYTLPPSRDELTKNQVSLTCLVKGFYPSDIAVEWESNGQPENNYKTTPPVLDSDGSFFLYSKLTVDKSRWQQGNVFSCSVMHEALHNHYTQKSLSLSPGK

SEQ ID NO: 102 - DNA, 4389 bp, Artificial Sequence
  FVIII 265
atgcaaatagagctctccacctgcttctttctgtgccttttgcgattctgctttagtggaggaggaggaggagccaccagaagatactacctgggtgcagtggaactgtcatgggactatatgcaaagtgatctcggtgagctgcctgtggacgcaagatttcctcctagagtgccaaaatcttttccattcaacacctcagtcgtgtacaaaaagactctgtttgtagaattcacggatcaccttttcaacatcgctaagccaaggccaccctggatgggtctgctaggtcctaccatccaggctgaggtttatgatacagtggtcattacacttaagaacatggcttcccatcctgtcagtcttcatgctgttggtgtatcctactggaaagcttctgagggagctgaatatgatgatcagaccagtcaaagggagaaagaagatgataaagtcttccctggtggaagccatacatatgtctggcaggtcctgaaagagaatggtccaatggcctctgacccactgtgccttacctactcatatctttctcatgtggacctggtaaaagacttgaattcaggcctcattggagccctactagtatgtagagaagggagtctggccaaggaaaagacacagaccttgcacaaatttatactactttttgctgtatttgatgaagggaaaagttggcactcagaaacaaagaactccttgatgcaggatagggatgctgcatctgctcgggcctggcctaaaatgcacacagtcaatggttatgtaaacaggtctctgccaggtctgattggatgccacaggaaatcagtctattggcatgtgattggaatgggcaccactcctgaagtgcactcaatattcctcgaaggtcacacatttcttgtgaggaaccatcgccaggcgtccttggaaatctcgccaataactttccttactgctcaaacactcttgatggaccttggacagtttctactgttttgtcatatctcttcccaccaacatgatggcatggaagcttatgtcaaagtagacagctgtccagaggaaccccaactacgaatgaaaaataatgaagaagcggaagactatgatgatgatcttactgattctgaaatggatgtggtcaggtttgatgatgacaactctccttcctttatccaaattcgctcagttgccaagaagcatcctaaaacttgggtacattacattgctgctgaagaggaggactgggactatgctcccttagtcctcgcccccgatgacagaagttataaaagtcaatatttgaacaatggccctcagcggattggtaggaagtacaaaaaagtccgatttatggcatacacagatgaaacctttaagactcgtgaagctattcagcatgaatcaggaatcttgggacctttactttatggggaagttggagacacactgttgattatatttaagaatcaagcaagcagaccatataacatctaccctcacggaatcactgatgtccgtcctttgtattcaaggagattaccaaaaggtgtaaaacatttgaaggattttccaattctgccaggagaaatattcaaatataaatggacagtgactgtagaagatgggccaactaaatcagatcctcggtgcctgacccgctattactctagtttcgttaatatggagagagatctagcttcaggactcattggccctctcctcatctgctacaaagaatctgtagatcaaagaggaaaccagataatgtcagacaagaggaatgtcatcctgttttctgtatttgatgagaaccgaagctggtacctcacagagaatatacaacgctttctccccaatccagctggagtgcagcttgaggatccagagttccaagcctccaacatcatgcacagcatcaatggctatgtttttgatagtttgcagttgtcagtttgtttgcatgaggtggcatactggtacattctaagcattggagcacagactgacttcctttctgtcttcttctctggatataccttcaaacacaaaatggtctatgaagacacactcaccctattcccattctcaggagaaactgtcttcatgtcgatggaaaacccaggtctatggattctggggtgccacaactcagactttcggaacagaggcatgaccgccttactgaaggtttctagttgtgacaagaacactggtgattattacgaggacagttatgaagatatttcagcatacttgctgagtaaaaacaatgccattgaaccaagaagcttctctcaaaacccaccagtcttgaaggcccatcaggccgaaataactcgtactactcttcagtcagatcaagaggaaattgactatgatgataccatatcagttgaaatgaagaaggaagattttgacatttatgatgaggatgaaaatcagagcccccgcagctttcaaaagaaaacacgacactattttattgctgcagtggagaggctctgggattatgggatgagtagctccccacatgttctaagaaacagggctcagagtggcagtgtccctcagttcaagaaagttgttttccaggaatttactgatggctcctttactcagcccttataccgtggagaactaaatgaacatttgggcctcctcggcccatatataagagcagaagttgaagataatatcatggtaactttcagaaatcaggcctctcgtccctattccttctattctagccttatttcttatgaggaagatcagaggcaaggagcagaacctagaaaaaactttgtcaagcctaatgaaaccaaaacttacttttggaaagtgcaacatcatatggcacccactaaagatgagtttgactgcaaagcctgggcttatttctctgatgttgacctggaaaaagatgtgcactcaggcctgattggaccccttctggtctgccacactaacacactgaaccctgctcatgggagacaagtgacagtacaggaatttgctctgtttttcaccatctttgatgagaccaaaagctggtacttcactgaaaatatggaaagaaactgcagggctccctgcaatatccagatggaagatcccacttttaaagagaattatcgcttccatgcaatcaatggctacataatggatacactacctggcttagtaatggctcaggatcaaaggattcgatggtatctgctcagcatgggcagcaatgaaaacatccattctattcatttcagtggacatgtgttcactgtacgaaaaaaagaggagtataaaatggcactgtacaatctctatccaggtgtttttgagacagtggaaatgttaccatccaaagctggaatttggcgggtggaatgccttattggcgagcatctacatgctgggatgagcacactttttctggtgtacagcaataagtgtcagactcccctgggaatggcttctggacacattagagattttcagattacagcttcaggacaatatggacagtgggccccaaagctggccagacttcattattccggatcaatcaatgcctggagcaccaaggagcccttttcttggatcaaggtggatctgttggcaccaatgattattcacggcatcaagacccagggtgcccgtcagaagttctccagcctctacatctctcagtttatcatcatgtatagtcttgatgggaagaagtggcagacttatcgaggaaattccactggaaccttaatggtcttctttggcaatgtggattcatctgggataaaacacaatatttttaaccctccaattattgctcgatacatccgtttgcacccaactcattatagcattcgcagcactcttcgcatggagttgatgggctgtgatttaaatagttgcagcatgccattgggaatggagagtaaagcaatatcagatgcacagattactgcttcatcctactttaccaatatgtttgccacctggtctccttcaaaagctcgacttcacctccaagggaggagtaatgcctggagacctcaggtgaataatccaaaagagtggctgcaagtggacttccagaagacaatgaaagtcacaggagtaactactcagggagtaaaatctctgcttaccagcatgtatgtgaaggagttcctcatctccagcagtcaagatggccatcagtggactctcttttttcagaatggcaaagtaaaggtttttcagggaaatcaagactccttcacacctgtggtgaactctctagacccaccgttactgactcgctaccttcgaattcacccccagagttgggtgcaccagattgccctgaggatggaggttctgggctgcgaggcacaggacctctactga

SEQ ID NO: 103 - protein, 1462 aa, Artificial Sequence
  FVIII 265
MQIELSTCFFLCLLRFCFSGGGGGATRRYYLGAVELSWDYMQSDLGELPVDARFPPRVPKSFPFNTSVVYKKTLFVEFTDHLFNIAKPRPPWMGLLGPTIQAEVYDTVVITLKNMASHPVSLHAVGVSYWKASEGAEYDDQTSQREKEDDKVFPGGSHTYVWQVLKENGPMASDPLCLTYSYLSHVDLVKDLNSGLIGALLVCREGSLAKEKTQTLHKFILLFAVFDEGKSWHSETKNSLMQDRDAASARAWPKMHTVNGYVNRSLPGLIGCHRKSVYWHVIGMGTTPEVHSIFLEGHTFLVRNHRQASLEISPITFLTAQTLLMDLGQFLLFCHISSHQHDGMEAYVKVDSCPEEPQLRMKNNEEAEDYDDDLTDSEMDVVRFDDDNSPSFIQIRSVAKKHPKTWVHYIAAEEEDWDYAPLVLAPDDRSYKSQYLNNGPQRIGRKYKKVRFMAYTDETFKTREAIQHESGILGPLLYGEVGDTLLIIFKNQASRPYNIYPHGITDVRPLYSRRLPKGVKHLKDFPILPGEIFKYKWTVTVEDGPTKSDPRCLTRYYSSFVNMERDLASGLIGPLLICYKESVDQRGNQIMSDKRNVILFSVFDENRSWYLTENIQRFLPNPAGVQLEDPEFQASNIMHSINGYVFDSLQLSVCLHEVAYWYILSIGAQTDFLSVFFSGYTFKHKMVYEDTLTLFPFSGETVFMSMENPGLWILGCHNSDFRNRGMTALLKVSSCDKNTGDYYEDSYEDISAYLLSKNNAIEPRSFSQNPPVLKAHQAEITRTTLQSDQEEIDYDDTISVEMKKEDFDIYDEDENQSPRSFQKKTRHYFIAAVERLWDYGMSSSPHVLRNRAQSGSVPQFKKVVFQEFTDGSFTQPLYRGELNEHLGLLGPYIRAEVEDNIMVTFRNQASRPYSFYSSLISYEEDQRQGAEPRKNFVKPNETKTYFWKVQHHMAPTKDEFDCKAWAYFSDVDLEKDVHSGLIGPLLVCHTNTLNPAHGRQVTVQEFALFFTIFDETKSWYFTENMERNCRAPCNIQMEDPTFKENYRFHAINGYIMDTLPGLVMAQDQRIRWYLLSMGSNENIHSIHFSGHVFTVRKKEEYKMALYNLYPGVFETVEMLPSKAGIWRVECLIGEHLHAGMSTLFLVYSNKCQTPLGMASGHIRDFQITASGQYGQWAPKLARLHYSGSINAWSTKEPFSWIKVDLLAPMIIHGIKTQGARQKFSSLYISQFIIMYSLDGKKWQTYRGNSTGTLMVFFGNVDSSGIKHNIFNPPIIARYIRLHPTHYSIRSTLRMELMGCDLNSCSMPLGMESKAISDAQITASSYFTNMFATWSPSKARLHLQGRSNAWRPQVNNPKEWLQVDFQKTMKVTGVTTQGVKSLLTSMYVKEFLISSSQDGHQWTLFFQNGKVKVFQGNQDSFTPVVNSLDPPLLTRYLRIHPQSWVHQIALRMEVLGCEAQDLY

SEQ ID NO: 104 - DNA, 5691 bp, Artificial Sequence
  FVIII198
atgcaaatagagctctccacctgcttctttctgtgccttttgcgattctgctttagtgccaccagaagatactacctgggtgcagtggaactgtcatgggactatatgcaaagtgatctcggtgagctgcctgtggacgcaagatttcctcctagagtgccaaaatcttttccattcaacacctcagtcgtgtacaaaaagactctgtttgtagaattcacggatcaccttttcaacatcgctaagccaaggccaccctggatgggtctgctaggtcctaccatccaggctgaggtttatgatacagtggtcattacacttaagaacatggcttcccatcctgtcagtcttcatgctgttggtgtatcctactggaaagcttctgagggagctgaatatgatgatcagaccagtcaaagggagaaagaagatgataaagtcttccctggtggaagccatacatatgtctggcaggtcctgaaagagaatggtccaatggcctctgacccactgtgccttacctactcatatctttctcatgtggacctggtaaaagacttgaattcaggcctcattggagccctactagtatgtagagaagggagtctggccaaggaaaagacacagaccttgcacaaatttatactactttttgctgtatttgatgaagggaaaagttggcactcagaaacaaagaactccttgatgcaggatagggatgctgcatctgctcgggcctggcctaaaatgcacacagtcaatggttatgtaaacaggtctctgccaggtctgattggatgccacaggaaatcagtctattggcatgtgattggaatgggcaccactcctgaagtgcactcaatattcctcgaaggtcacacatttcttgtgaggaaccatcgccaggcgtccttggaaatctcgccaataactttccttactgctcaaacactcttgatggaccttggacagtttctactgttttgtcatatctcttcccaccaacatgatggcatggaagcttatgtcaaagtagacagctgtccagaggaaccccaactacgaatgaaaaataatgaagaagcggaagactatgatgatgatcttactgattctgaaatggatgtggtcaggtttgatgatgacaactctccttcctttatccaaattcgctcagttgccaagaagcatcctaaaacttgggtacattacattgctgctgaagaggaggactgggactatgctcccttagtcctcgcccccgatgacagaagttataaaagtcaatatttgaacaatggccctcagcggattggtaggaagtacaaaaaagtccgatttatggcatacacagatgaaacctttaagactcgtgaagctattcagcatgaatcaggaatcttgggacctttactttatggggaagttggagacacactgttgattatatttaagaatcaagcaagcagaccatataacatctaccctcacggaatcactgatgtccgtcctttgtattcaaggagattaccaaaaggtgtaaaacatttgaaggattttccaattctgccaggagaaatattcaaatataaatggacagtgactgtagaagatgggccaactaaatcagatcctcggtgcctgacccgctattactctagtttcgttaatatggagagagatctagcttcaggactcattggccctctcctcatctgctacaaagaatctgtagatcaaagaggaaaccagataatgtcagacaagaggaatgtcatcctgttttctgtatttgatgagaaccgaagctggtacctcacagagaatatacaacgctttctccccaatccagctggagtgcagcttgaggatccagagttccaagcctccaacatcatgcacagcatcaatggctatgtttttgatagtttgcagttgtcagtttgtttgcatgaggtggcatactggtacattctaagcattggagcacagactgacttcctttctgtcttcttctctggatataccttcaaacacaaaatggtctatgaagacacactcaccctattcccattctcaggagaaactgtcttcatgtcgatggaaaacccaggtctatggattctggggtgccacaactcagactttcggaacagaggcatgaccgccttactgaaggtttctagttgtgacaagaacactggtgattattacgaggacagttatgaagatatttcagcatacttgctgagtaaaaacaatgccattgaaccaagaagcttctctcagaattcaagacaccctagcactaggcaaaagcaatttaatgccaccacaattccagaaaatgacatagagaagactgacccttggtttgcacacagaacacctatgcctaaaatacaaaatgtctcctctagtgatttgttgatgctcttgcgacagagtcctactccacatgggctatccttatctgatctccaagaagccaaatatgagactttttctgatgatccatcacctggagcaatagacagtaataacagcctgtctgaaatgacacacttcaggccacagctccatcacagtggggacatggtatttacccctgagtcaggcctccaattaagattaaatgagaaactggggacaactgcagcaacagagttgaagaaacttgatttcaaagtttctagtacatcaaataatctgatttcaacaattccatcagacaatttggcagcaggtactgataatacaagttccttaggacccccaagtatgccagttcattatgatagtcaattagataccactctatttggcaaaaagtcatctccccttactgagtctggtggacctctgagcttgagtgaagaaaataatgattcaaagttgttagaatcaggtttaatgaatagccaagaaagttcatggggaaaaaatgtatcgtcagaaataactcgtactactcttcagtcagatcaagaggaaattgactatgatgataccatatcagttgaaatgaagaaggaagattttgacatttatgatgaggatgaaaatcagagcccccgcagctttcaaaagaaaacacgacactattttattgctgcagtggagaggctctgggattatgggatgagtagctccccacatgttctaagaaacagggctcagagtggcagtgtccctcagttcaagaaagttgttttccaggaatttactgatggctcctttactcagcccttataccgtggagaactaaatgaacatttgggactcctggggccatatataagagcagaagttgaagataatatcatggtaactttcagaaatcaggcctctcgtccctattccttctattctagccttatttcttatgaggaagatcagaggcaaggagcagaacctagaaaaaactttgtcaagcctaatgaaaccaaaacttacttttggaaagtgcaacatcatatggcacccactaaagatgagtttgactgcaaagcctgggcttatttctctgatgttgacctggaaaaagatgtgcactcaggcctgattggaccccttctggtctgccacactaacacactgaaccctgctcatgggagacaagtgacagtacaggaatttgctctgtttttcaccatctttgatgagaccaaaagctggtacttcactgaaaatatggaaagaaactgcagggctccctgcaatatccagatggaagatcccacttttaaagagaattatcgcttccatgcaatcaatggctacataatggatacactacctggcttagtaatggctcaggatcaaaggattcgatggtatctgctcagcatgggcagcaatgaaaacatccattctattcatttcagtggacatgtgttcactgtacgaaaaaaagaggagtataaaatggcactgtacaatctctatccaggtgtttttgagacagtggaaatgttaccatccaaagctggaatttggcgggtggaatgccttattggcgagcatctacatgctgggatgagcacactttttctggtgtacagcaataagtgtcagactcccctgggaatggcttctggacacattagagattttcagattacagcttcaggacaatatggacagtgggccccaaagctggccagacttcattattccggatcaatcaatgcctggagcaccaaggagcccttttcttggatcaaggtggatctgttggcaccaatgattattcacggcatcaagacccagggtgcccgtcagaagttctccagcctctacatctctcagtttatcatcatgtatagtcttgatgggaagaagtggcagacttatcgaggaaattccactggaaccttaatggtcttctttggcaatgtggattcatctgggataaaacacaatatttttaaccctccaattattgctcgatacatccgtttgcacccaactcattatagcattcgcagcactcttcgcatggagttgatgggctgtgatttaaatagttgcagcatgccattgggaatggagagtaaagcaatatcagatgcacagattactgcttcatcctactttaccaatatgtttgccacctggtctccttcaaaagctcgacttcacctccaagggaggagtaatgcctggagacctcaggtgaataatccaaaagagtggctgcaagtggacttccagaagacaatgaaagtcacaggagtaactactcagggagtaaaatctctgcttaccagcatgtatgtgaaggagttcctcatctccagcagtcaagatggccatcagtggactctcttttttcagaatggcaaagtaaaggtttttcagggaaatcaagactccttcacacctgtggtgaactctctagacccaccgttactgactcgctaccttcgaattcacccccagagttgggtgcaccagattgccctgaggatggaggttctgggctgcgaggcacaggacctctacgacaaaactcacacatgcccaccgtgcccagctccagaactcctgggcggaccgtcagtcttcctcttccccccaaaacccaaggacaccctcatgatctcccggacccctgaggtcacatgcgtggtggtggacgtgagccacgaagaccctgaggtcaagttcaactggtacgtggacggcgtggaggtgcataatgccaagacaaagccgcgggaggagcagtacaacagcacgtaccgtgtggtcagcgtcctcaccgtcctgcaccaggactggctgaatggcaaggagtacaagtgcaaggtctccaacaaagccctcccagcccccatcgagaaaaccatctccaaagccaaagggcagccccgagaaccacaggtgtacaccctgcccccatcccgggatgagctgaccaagaaccaggtcagcctgacctgcctggtcaaaggcttctatcccagcgacatcgccgtggagtgggagagcaatgggcagccggagaacaactacaagaccacgcctcccgtgttggactccgacggctccttcttcctctacagcaagctcaccgtggacaagagcaggtggcagcaggggaacgtcttctcatgctccgtgatgcatgaggctctgcacaaccactacacgcagaagagcctctccctgtctccgggtaaatga

SEQ ID NO: 105 - protein, 1896 aa, Artificial Sequence
  FVIII 198
MQIELSTCFFLCLLRFCFSATRRYYLGAVELSWDYMQSDLGELPVDARFPPRVPKSFPFNTSVVYKKTLFVEFTDHLFNIAKPRPPWMGLLGPTIQAEVYDTVVITLKNMASHPVSLHAVGVSYWKASEGAEYDDQTSQREKEDDKVFPGGSHTYVWQVLKENGPMASDPLCLTYSYLSHVDLVKDLNSGLIGALLVCREGSLAKEKTQTLHKFILLFAVFDEGKSWHSETKNSLMQDRDAASARAWPKMHTVNGYVNRSLPGLIGCHRKSVYWHVIGMGTTPEVHSIFLEGHTFLVRNHRQASLEISPITFLTAQTLLMDLGQFLLFCHISSHQHDGMEAYVKVDSCPEEPQLRMKNNEEAEDYDDDLTDSEMDVVRFDDDNSPSFIQIRSVAKKHPKTWVHYIAAEEEDWDYAPLVLAPDDRSYKSQYLNNGPQRIGRKYKKVRFMAYTDETFKTREAIQHESGILGPLLYGEVGDTLLIIFKNQASRPYNIYPHGITDVRPLYSRRLPKGVKHLKDFPILPGEIFKYKWTVTVEDGPTKSDPRCLTRYYSSFVNMERDLASGLIGPLLICYKESVDQRGNQIMSDKRNVILFSVFDENRSWYLTENIQRFLPNPAGVQLEDPEFQASNIMHSINGYVFDSLQLSVCLHEVAYWYILSIGAQTDFLSVFFSGYTFKHKMVYEDTLTLFPFSGETVFMSMENPGLWILGCHNSDFRNRGMTALLKVSSCDKNTGDYYEDSYEDISAYLLSKNNAIEPRSFSQNSRHPSTRQKQFNATTIPENDIEKTDPWFAHRTPMPKIQNVSSSDLLMLLRQSPTPHGLSLSDLQEAKYETFSDDPSPGAIDSNNSLSEMTHFRPQLHHSGDMVFTPESGLQLRLNEKLGTTAATELKKLDFKVSSTSNNLISTIPSDNLAAGTDNTSSLGPPSMPVHYDSQLDTTLFGKKSSPLTESGGPLSLSEENNDSKLLESGLMNSQESSWGKNVSSEITRTTLQSDQEEIDYDDTISVEMKKEDFDIYDEDENQSPRSFQKKTRHYFIAAVERLWDYGMSSSPHVLRNRAQSGSVPQFKKVVFQEFTDGSFTQPLYRGELNEHLGLLGPYIRAEVEDNIMVTFRNQASRPYSFYSSLISYEEDQRQGAEPRKNFVKPNETKTYFWKVQHHMAPTKDEFDCKAWAYFSDVDLEKDVHSGLIGPLLVCHTNTLNPAHGRQVTVQEFALFFTIFDETKSWYFTENMERNCRAPCNIQMEDPTFKENYRFHAINGYIMDTLPGLVMAQDQRIRWYLLSMGSNENIHSIHFSGHVFTVRKKEEYKMALYNLYPGVFETVEMLPSKAGIWRVECLIGEHLHAGMSTLFLVYSNKCQTPLGMASGHIRDFQITASGQYGQWAPKLARLHYSGSINAWSTKEPFSWIKVDLLAPMIIHGIKTQGARQKFSSLYISQFIIMYSLDGKKWQTYRGNSTGTLMVFFGNVDSSGIKHNIFNPPIIARYIRLHPTHYSIRSTLRMELMGCDLNSCSMPLGMESKAISDAQITASSYFTNMFATWSPSKARLHLQGRSNAWRPQVNNPKEWLQVDFQKTMKVTGVTTQGVKSLLTSMYVKEFLISSSQDGHQWTLFFQNGKVKVFQGNQDSFTPVVNSLDPPLLTRYLRIHPQSWVHQIALRMEVLGCEAQDLYDKTHTCPPCPAPELLGGPSVFLFPPKPKDTLMISRTPEVTCVVVDVSHEDPEVKFNWYVDGVEVHNAKTKPREEQYNSTYRVVSVLTVLHQDWLNGKEYKCKVSNKALPAPIEKTISKAKGQPREPQVYTLPPSRDELTKNQVSLTCLVKGFYPSDIAVEWESNGQPENNYKTTPPVLDSDGSFFLYSKLTVDKSRWQQGNVFSCSVMHEALHNHYTQKSLSLSPGK

SEQ ID NO: 106 - protein, 5 aa, Artificial Sequence
  sortase recognition motif
  variant (3)..(3): Xaa can be any naturally occurring amino acid
LPXTG

SEQ ID NO: 107 - protein, 10 aa, Artificial Sequence
  cysteine containing peptide
GGGSGCGGGS

SEQ ID NO: 108 - DNA, 4548 bp, Artificial Sequence
  VWF 031
atgattcctgccagatttgccggggtgctgcttgctctggccctcattttgccagggaccctttgtgcagaaggaactcgcggcaggtcatccacggcccgatgcagccttttcggaagtgacttcgtcaacacctttgatgggagcatgtacagctttgcgggatactgcagttacctcctggcagggggctgccagaaacgctccttctcgattattggggacttccagaatggcaagagagtgagcctctccgtgtatcttggggaattttttgacatccatttgtttgtcaatggtaccgtgacacagggggaccaaagagtctccatgccctatgcctccaaagggctgtatctagaaactgaggctgggtactacaagctgtccggtgaggcctatggctttgtggccaggatcgatggcagcggcaactttcaagtcctgctgtcagacagatacttcaacaagacctgcgggctgtgtggcaactttaacatctttgctgaagatgactttatgacccaagaagggaccttgacctcggacccttatgactttgccaactcatgggctctgagcagtggagaacagtggtgtgaacgggcatctcctcccagcagctcatgcaacatctcctctggggaaatgcagaagggcctgtgggagcagtgccagcttctgaagagcacctcggtgtttgcccgctgccaccctctggtggaccccgagccttttgtggccctgtgtgagaagactttgtgtgagtgtgctggggggctggagtgcgcctgccctgccctcctggagtacgcccggacctgtgcccaggagggaatggtgctgtacggctggaccgaccacagcgcgtgcagcccagtgtgccctgctggtatggagtataggcagtgtgtgtccccttgcgccaggacctgccagagcctgcacatcaatgaaatgtgtcaggagcgatgcgtggatggctgcagctgccctgagggacagctcctggatgaaggcctctgcgtggagagcaccgagtgtccctgcgtgcattccggaaagcgctaccctcccggcacctccctctctcgagactgcaacacctgcatttgccgaaacagccagtggatctgcagcaatgaagaatgtccaggggagtgccttgtcactggtcaatcccacttcaagagctttgacaacagatacttcaccttcagtgggatctgccagtacctgctggcccgggattgccaggaccactccttctccattgtcattgagactgtccagtgtgctgatgaccgcgacgctgtgtgcacccgctccgtcaccgtccggctgcctggcctgcacaacagccttgtgaaactgaagcatggggcaggagttgccatggatggccaggacatccagctccccctcctgaaaggtgacctccgcatccagcatacagtgacggcctccgtgcgcctcagctacggggaggacctgcagatggactgggatggccgcgggaggctgctggtgaagctgtcccccgtctatgccgggaagacctgcggcctgtgtgggaattacaatggcaaccagggcgacgacttccttaccccctctgggctggcggagccccgggtggaggacttcgggaacgcctggaagctgcacggggactgccaggacctgcagaagcagcacagcgatccctgcgccctcaacccgcgcatgaccaggttctccgaggaggcgtgcgcggtcctgacgtcccccacattcgaggcctgccatcgtgccgtcagcccgctgccctacctgcggaactgccgctacgacgtgtgctcctgctcggacggccgcgagtgcctgtgcggcgccctggccagctatgccgcggcctgcgcggggagaggcgtgcgcgtcgcgtggcgcgagccaggccgctgtgagctgaactgcccgaaaggccaggtgtacctgcagtgcgggaccccctgcaacctgacctgccgctctctctcttacccggatgaggaatgcaatgaggcctgcctggagggctgcttctgccccccagggctctacatggatgagaggggggactgcgtgcccaaggcccagtgcccctgttactatgacggtgagatcttccagccagaagacatcttctcagaccatcacaccatgtgctactgtgaggatggcttcatgcactgtaccatgagtggagtccccggaagcttgctgcctgacgctgtcctcagcagtcccctgtctcatcgcagcaaaaggagcctatcctgtcggccccccatggtcaagctggtgtgtcccgctgacaacctgcgggctgaagggctcgagtgtaccaaaacgtgccagaactatgacctggagtgcatgagcatgggctgtgtctctggctgcctctgccccccgggcatggtccggcatgagaacagatgtgtggccctggaaaggtgtccctgcttccatcagggcaaggagtatgcccctggagaaacagtgaagattggctgcaacacttgtgtctgtcgggaccggaagtggaactgcacagaccatgtgtgtgatgccacgtgctccacgatcggcatggcccactacctcaccttcgacgggctcaaatacctgttccccggggagtgccagtacgttctggtgcaggattactgcggcagtaaccctgggacctttcggatcctagtggggaataagggatgcagccacccctcagtgaaatgcaagaaacgggtcaccatcctggtggagggaggagagattgagctgtttgacggggaggtgaatgtgaagaggcccatgaaggatgagactcactttgaggtggtggagtctggccggtacatcattctgctgctgggcaaagccctctccgtggtctgggaccgccacctgagcatctccgtggtcctgaagcagacataccaggagaaagtgtgtggcctgtgtgggaattttgatggcatccagaacaatgacctcaccagcagcaacctccaagtggaggaagaccctgtggactttgggaactcctggaaagtgagctcgcagtgtgctgacaccagaaaagtgcctctggactcatcccctgccacctgccataacaacatcatgaagcagacgatggtggattcctcctgtagaatccttaccagtgacgtcttccaggactgcaacaagctggtggaccccgagccatatctggatgtctgcatttacgacacctgctcctgtgagtccattggggactgcgccgcattctgcgacaccattgctgcctatgcccacgtgtgtgcccagcatggcaaggtggtgacctggaggacggccacattgtgcccccagagctgcgaggagaggaatctccgggagaacgggtatgaggctgagtggcgctataacagctgtgcacctgcctgtcaagtcacgtgtcagcaccctgagccactggcctgccctgtgcagtgtgtggagggctgccatgcccactgccctccagggaaaatcctggatgagcttttgcagacctgcgttgaccctgaagactgtccagtgtgtgaggtggctggccggcgttttgcctcaggaaagaaagtcaccttgaatcccagtgaccctgagcactgccagatttgccactgtgatgttgtcaacctcacctgtgaagcctgccaggagccgatatctggcggtggaggttccggtggcgggggatccggcggtggaggttccggcggtggaggttccggtggcgggggatccggtggcgggggatccctggtcccccggggcagcggcggtggaggttccggtggcgggggatccgacaaaactcacacatgcccaccgtgcccagctccagaactcctgggcggaccgtcagtcttcctcttccccccaaaacccaaggacaccctcatgatctcccggacccctgaggtcacatgcgtggtggtggacgtgagccacgaagaccctgaggtcaagttcaactggtacgtggacggcgtggaggtgcataatgccaagacaaagccgcgggaggagcagtacaacagcacgtaccgtgtggtcagcgtcctcaccgtcctgcaccaggactggctgaatggcaaggagtacaagtgcaaggtctccaacaaagccctcccagcccccatcgagaaaaccatctccaaagccaaagggcagccccgagaaccacaggtgtacaccctgcccccatcccgggatgagctgaccaagaaccaggtcagcctgacctgcctggtcaaaggcttctatcccagcgacatcgccgtggagtgggagagcaatgggcagccggagaacaactacaagaccacgcctcccgtgttggactccgacggctccttcttcctctacagcaagctcaccgtggacaagagcaggtggcagcaggggaacgtcttctcatgctccgtgatgcatgaggctctgcacaaccactacacgcagaagagcctctccctgtctccgggtaaatga

SEQ ID NO: 109 - protein, 1515 aa, Artificial Sequence
  VWF 031
MIPARFAGVLLALALILPGTLCAEGTRGRSSTARCSLFGSDFVNTFDGSMYSFAGYCSYLLAGGCQKRSFSIIGDFQNGKRVSLSVYLGEFFDIHLFVNGTVTQGDQRVSMPYASKGLYLETEAGYYKLSGEAYGFVARIDGSGNFQVLLSDRYFNKTCGLCGNFNIFAEDDFMTQEGTLTSDPYDFANSWALSSGEQWCERASPPSSSCNISSGEMQKGLWEQCQLLKSTSVFARCHPLVDPEPFVALCEKTLCECAGGLECACPALLEYARTCAQEGMVLYGWTDHSACSPVCPAGMEYRQCVSPCARTCQSLHINEMCQERCVDGCSCPEGQLLDEGLCVESTECPCVHSGKRYPPGTSLSRDCNTCICRNSQWICSNEECPGECLVTGQSHFKSFDNRYFTFSGICQYLLARDCQDHSFSIVIETVQCADDRDAVCTRSVTVRLPGLHNSLVKLKHGAGVAMDGQDIQLPLLKGDLRIQHTVTASVRLSYGEDLQMDWDGRGRLLVKLSPVYAGKTCGLCGNYNGNQGDDFLTPSGLAEPRVEDFGNAWKLHGDCQDLQKQHSDPCALNPRMTRFSEEACAVLTSPTFEACHRAVSPLPYLRNCRYDVCSCSDGRECLCGALASYAAACAGRGVRVAWREPGRCELNCPKGQVYLQCGTPCNLTCRSLSYPDEECNEACLEGCFCPPGLYMDERGDCVPKAQCPCYYDGEIFQPEDIFSDHHTMCYCEDGFMHCTMSGVPGSLLPDAVLSSPLSHRSKRSLSCRPPMVKLVCPADNLRAEGLECTKTCQNYDLECMSMGCVSGCLCPPGMVRHENRCVALERCPCFHQGKEYAPGETVKIGCNTCVCRDRKWNCTDHVCDATCSTIGMAHYLTFDGLKYLFPGECQYVLVQDYCGSNPGTFRILVGNKGCSHPSVKCKKRVTILVEGGEIELFDGEVNVKRPMKDETHFEVVESGRYIILLLGKALSVVWDRHLSISVVLKQTYQEKVCGLCGNFDGIQNNDLTSSNLQVEEDPVDFGNSWKVSSQCADTRKVPLDSSPATCHNNIMKQTMVDSSCRILTSDVFQDCNKLVDPEPYLDVCIYDTCSCESIGDCAAFCDTIAAYAHVCAQHGKVVTWRTATLCPQSCEERNLRENGYEAEWRYNSCAPACQVTCQHPEPLACPVQCVEGCHAHCPPGKILDELLQTCVDPEDCPVCEVAGRRFASGKKVTLNPSDPEHCQICHCDVVNLTCEACQEPISGGGGSGGGGSGGGGSGGGGSGGGGSGGGGSLVPRGSGGGGSGGGGSDKTHTCPPCPAPELLGGPSVFLFPPKPKDTLMISRTPEVTCVVVDVSHEDPEVKFNWYVDGVEVHNAKTKPREEQYNSTYRVVSVLTVLHQDWLNGKEYKCKVSNKALPAPIEKTISKAKGQPREPQVYTLPPSRDELTKNQVSLTCLVKGFYPSDIAVEWESNGQPENNYKTTPPVLDSDGSFFLYSKLTVDKSRWQQGNVFSCSVMHEALHNHYTQKSLSLSPGK

SEQ ID NO: 110 - protein, 40 aa, Artificial Sequence
  linker
  REPEAT (1)..(5): Gly-Gly-Gly-Gly-Ser repeat
GGGGSGGGGSGGGGSGGGGSGGGGSGGGGSGGGGSGGGGS

SEQ ID NO: 111 - DNA, 62 bp, Artificial Sequence
  ESC54-VWF forward with BsiW1 site
cgcttcgcgacgtacggccgccaccatgattcctgccagatttgccggggtgctgcttgctc

SEQ ID NO: 112 - DNA, 60 bp, Artificial Sequence
  ESC 124 - D1D2 cloning oligo with Not1 site-reverse
ctagactcgagcggccgctcaccttttgctgcgatgagacaggggactgctgaggacagc

SEQ ID NO: 113 - DNA, 2289 bp, Artificial Sequence
  VWF 053 (VWF D1D2-propeptide)
atgattcctgccagatttgccggggtgctgcttgctctggccctcattttgccagggaccctttgtgcagaaggaactcgcggcaggtcatccacggcccgatgcagccttttcggaagtgacttcgtcaacacctttgatgggagcatgtacagctttgcgggatactgcagttacctcctggcagggggctgccagaaacgctccttctcgattattggggacttccagaatggcaagagagtgagcctctccgtgtatcttggggaattttttgacatccatttgtttgtcaatggtaccgtgacacagggggaccaaagagtctccatgccctatgcctccaaagggctgtatctagaaactgaggctgggtactacaagctgtccggtgaggcctatggctttgtggccaggatcgatggcagcggcaactttcaagtcctgctgtcagacagatacttcaacaagacctgcgggctgtgtggcaactttaacatctttgctgaagatgactttatgacccaagaagggaccttgacctcggacccttatgactttgccaactcatgggctctgagcagtggagaacagtggtgtgaacgggcatctcctcccagcagctcatgcaacatctcctctggggaaatgcagaagggcctgtgggagcagtgccagcttctgaagagcacctcggtgtttgcccgctgccaccctctggtggaccccgagccttttgtggccctgtgtgagaagactttgtgtgagtgtgctggggggctggagtgcgcctgccctgccctcctggagtacgcccggacctgtgcccaggagggaatggtgctgtacggctggaccgaccacagcgcgtgcagcccagtgtgccctgctggtatggagtataggcagtgtgtgtccccttgcgccaggacctgccagagcctgcacatcaatgaaatgtgtcaggagcgatgcgtggatggctgcagctgccctgagggacagctcctggatgaaggcctctgcgtggagagcaccgagtgtccctgcgtgcattccggaaagcgctaccctcccggcacctccctctctcgagactgcaacacctgcatttgccgaaacagccagtggatctgcagcaatgaagaatgtccaggggagtgccttgtcactggtcaatcccacttcaagagctttgacaacagatacttcaccttcagtgggatctgccagtacctgctggcccgggattgccaggaccactccttctccattgtcattgagactgtccagtgtgctgatgaccgcgacgctgtgtgcacccgctccgtcaccgtccggctgcctggcctgcacaacagccttgtgaaactgaagcatggggcaggagttgccatggatggccaggacatccagctccccctcctgaaaggtgacctccgcatccagcatacagtgacggcctccgtgcgcctcagctacggggaggacctgcagatggactgggatggccgcgggaggctgctggtgaagctgtcccccgtctatgccgggaagacctgcggcctgtgtgggaattacaatggcaaccagggcgacgacttccttaccccctctgggctggcggagccccgggtggaggacttcgggaacgcctggaagctgcacggggactgccaggacctgcagaagcagcacagcgatccctgcgccctcaacccgcgcatgaccaggttctccgaggaggcgtgcgcggtcctgacgtcccccacattcgaggcctgccatcgtgccgtcagcccgctgccctacctgcggaactgccgctacgacgtgtgctcctgctcggacggccgcgagtgcctgtgcggcgccctggccagctatgccgcggcctgcgcggggagaggcgtgcgcgtcgcgtggcgcgagccaggccgctgtgagctgaactgcccgaaaggccaggtgtacctgcagtgcgggaccccctgcaacctgacctgccgctctctctcttacccggatgaggaatgcaatgaggcctgcctggagggctgcttctgccccccagggctctacatggatgagaggggggactgcgtgcccaaggcccagtgcccctgttactatgacggtgagatcttccagccagaagacatcttctcagaccatcacaccatgtgctactgtgaggatggcttcatgcactgtaccatgagtggagtccccggaagcttgctgcctgacgctgtcctcagcagtcccctgtctcatcgcagcaaaagg

SEQ ID NO: 114 - protein, 763 aa, Artificial Sequence
  VWF 053 (VWF D1D2-Propeptide)
MIPARFAGVLLALALILPGTLCAEGTRGRSSTARCSLFGSDFVNTFDGSMYSFAGYCSYLLAGGCQKRSFSIIGDFQNGKRVSLSVYLGEFFDIHLFVNGTVTQGDQRVSMPYASKGLYLETEAGYYKLSGEAYGFVARIDGSGNFQVLLSDRYFNKTCGLCGNFNIFAEDDFMTQEGTLTSDPYDFANSWALSSGEQWCERASPPSSSCNISSGEMQKGLWEQCQLLKSTSVFARCHPLVDPEPFVALCEKTLCECAGGLECACPALLEYARTCAQEGMVLYGWTDHSACSPVCPAGMEYRQCVSPCARTCQSLHINEMCQERCVDGCSCPEGQLLDEGLCVESTECPCVHSGKRYPPGTSLSRDCNTCICRNSQWICSNEECPGECLVTGQSHFKSFDNRYFTFSGICQYLLARDCQDHSFSIVIETVQCADDRDAVCTRSVTVRLPGLHNSLVKLKHGAGVAMDGQDIQLPLLKGDLRIQHTVTASVRLSYGEDLQMDWDGRGRLLVKLSPVYAGKTCGLCGNYNGNQGDDFLTPSGLAEPRVEDFGNAWKLHGDCQDLQKQHSDPCALNPRMTRFSEEACAVLTSPTFEACHRAVSPLPYLRNCRYDVCSCSDGRECLCGALASYAAACAGRGVRVAWREPGRCELNCPKGQVYLQCGTPCNLTCRSLSYPDEECNEACLEGCFCPPGLYMDERGDCVPKAQCPCYYDGEIFQPEDIFSDHHTMCYCEDGFMHCTMSGVPGSLLPDAVLSSPLSHRSKR